European Patent Application EP 4 706 776 A2, published March 11, 2026. Title: METHOD AND COMPOSITIONS FOR CELLULAR IMMUNOTHERAPY. Applicant: Fred Hutchinson Cancer Center. Application EP 25150326.4, filed August 20, 2013. The sequence listing filed with the application follows.

SEQUENCE LISTING (114 sequences)

SEQ ID NO: 1 - skipped

SEQ ID NO: 2 - DNA, 66 bp, synthetic construct
  misc_feature 1..66: note = Synthetic
  source 1..66: mol_type = other DNA
atgctgctgctggtgaccagcctgctgctgtgcgagctgccccaccccgcctttctgctgatcccc

SEQ ID NO: 3 - DNA, 735 bp, synthetic construct
  misc_feature 1..735: note = Synthetic
  source 1..735: mol_type = other DNA
gacatccagatgacccagaccacctccagcctgagcgccagcctgggcgaccgggtgaccatcagctgccgggccagccaggacatcagcaagtacctgaactggtatcagcagaagcccgacggcaccgtcaagctgctgatctaccacaccagccggctgcacagcggcgtgcccagccggtttagcggcagcggctccggcaccgactacagcctgaccatctccaacctggaacaggaagatatcgccacctacttttgccagcagggcaacacactgccctacacctttggcggcggaacaaagctggaaatcaccggcagcacctccggcagcggcaagcctggcagcggcgagggcagcaccaagggcgaggtgaagctgcaggaaagcggccctggcctggtggcccccagccagagcctgagcgtgacctgcaccgtgagcggcgtgagcctgcccgactacggcgtgagctggatccggcagccccccaggaagggcctggaatggctgggcgtgatctggggcagcgagaccacctactacaacagcgccctgaagagccggctgaccatcatcaaggacaacagcaagagccaggtgttcctgaagatgaacagcctgcagaccgacgacaccgccatctactactgcgccaagcactactactacggcggcagctacgccatggactactggggccagggcaccagcgtgaccgtgagcagc

SEQ ID NO: 4 - DNA, 36 bp, synthetic construct
  misc_feature 1..36: note = Synthetic
  source 1..36: mol_type = other DNA
gaatctaagtacggaccgccctgccccccttgccct

SEQ ID NO: 5 - DNA, 84 bp, synthetic construct
  misc_feature 1..84: note = Synthetic
  source 1..84: mol_type = other DNA
atgttctgggtgctggtggtggtcggaggcgtgctggcctgctacagcctgctggtcaccgtggccttcatcatcttttgggtg

SEQ ID NO: 6 - DNA, 126 bp, synthetic construct
  misc_feature 1..126: note = Synthetic
  source 1..126: mol_type = other DNA
aaacggggcagaaagaaactcctgtatatattcaaacaaccatttatgagaccagtacaaactactcaagaggaagatggctgtagctgccgatttccagaagaagaagaaggaggatgtgaactg

SEQ ID NO: 7 - DNA, 336 bp, synthetic construct
  misc_feature 1..336: note = Synthetic
  source 1..336: mol_type = other DNA
cgggtgaagttcagcagaagcgccgacgcccctgcctaccagcagggccagaatcagctgtacaacgagctgaacctgggcagaagggaagagtacgacgtcctggataagcggagaggccgggaccctgagatgggcggcaagcctcggcggaagaacccccaggaaggcctgtataacgaactgcagaaagacaagatggccgaggcctacagcgagatcggcatgaagggcgagcggaggcggggcaagggccacgacggcctgtatcagggcctgtccaccgccaccaaggatacctacgacgccctgcacatgcaggccctgcccccaagg

SEQ ID NO: 8 - DNA, 72 bp, synthetic construct
  misc_feature 1..72: note = Synthetic
  source 1..72: mol_type = other DNA
ctcgagggcggcggagagggcagaggaagtcttctaacatgcggtgacgtggaggagaatcccggccctagg

SEQ ID NO: 9 - DNA, 1074 bp, synthetic construct
  misc_feature 1..1074: note = Synthetic
  source 1..1074: mol_type = other DNA
atgcttctcctggtgacaagccttctgctctgtgagttaccacacccagcattcctcctgatcccacgcaaagtgtgtaacggaataggtattggtgaatttaaagactcactctccataaatgctacgaatattaaacacttcaaaaactgcacctccatcagtggcgatctccacatcctgccggtggcatttaggggtgactccttcacacatactcctcctctggatccacaggaactggatattctgaaaaccgtaaaggaaatcacagggtttttgctgattcaggcttggcctgaaaacaggacggacctccatgcctttgagaacctagaaatcatacgcggcaggaccaagcaacatggtcagttttctcttgcagtcgtcagcctgaacataacatccttgggattacgctccctcaaggagataagtgatggagatgtgataatttcaggaaacaaaaatttgtgctatgcaaatacaataaactggaaaaaactgtttgggacctccggtcagaaaaccaaaattataagcaacagaggtgaaaacagctgcaaggccacaggccaggtctgccatgccttgtgctcccccgagggctgctggggcccggagcccagggactgcgtctcttgccggaatgtcagccgaggcagggaatgcgtggacaagtgcaaccttctggagggtgagccaagggagtttgtggagaactctgagtgcatacagtgccacccagagtgcctgcctcaggccatgaacatcacctgcacaggacggggaccagacaactgtatccagtgtgcccactacattgacggcccccactgcgtcaagacctgcccggcaggagtcatgggagaaaacaacaccctggtctggaagtacgcagacgccggccatgtgtgccacctgtgccatccaaactgcacctacggatgcactgggccaggtcttgaaggctgtccaacgaatgggcctaagatcccgtccatcgccactgggatggtgggggccctcctcttgctgctggtggtggccctggggatcggcctcttcatgtga

SEQ ID NO: 10 - DNA, 2529 bp, synthetic construct
  misc_feature 1..2529: note = Synthetic
  source 1..2529: mol_type = other DNA
atgctgctgctggtgaccagcctgctgctgtgcgagctgccccaccccgcctttctgctgatccccgacatccagatgacccagaccacctccagcctgagcgccagcctgggcgaccgggtgaccatcagctgccgggccagccaggacatcagcaagtacctgaactggtatcagcagaagcccgacggcaccgtcaagctgctgatctaccacaccagccggctgcacagcggcgtgcccagccggtttagcggcagcggctccggcaccgactacagcctgaccatctccaacctggaacaggaagatatcgccacctacttttgccagcagggcaacacactgccctacacctttggcggcggaacaaagctggaaatcaccggcagcacctccggcagcggcaagcctggcagcggcgagggcagcaccaagggcgaggtgaagctgcaggaaagcggccctggcctggtggcccccagccagagcctgagcgtgacctgcaccgtgagcggcgtgagcctgcccgactacggcgtgagctggatccggcagccccccaggaagggcctggaatggctgggcgtgatctggggcagcgagaccacctactacaacagcgccctgaagagccggctgaccatcatcaaggacaacagcaagagccaggtgttcctgaagatgaacagcctgcagaccgacgacaccgccatctactactgcgccaagcactactactacggcggcagctacgccatggactactggggccagggcaccagcgtgaccgtgagcagcgagagcaagtacggaccgccctgccccccttgccctatgttctgggtgctggtggtggtcggaggcgtgctggcctgctacagcctgctggtcaccgtggccttcatcatcttttgggtgaaacggggcagaaagaaactcctgtatatattcaaacaaccatttatgagaccagtacaaactactcaagaggaagatggctgtagctgccgatttccagaagaagaagaaggaggatgtgaactgcgggtgaagttcagcagaagcgccgacgcccctgcctaccagcagggccagaatcagctgtacaacgagctgaacctgggcagaagggaagagtacgacgtcctggataagcggagaggccgggaccctgagatgggcggcaagcctcggcggaagaacccccaggaaggcctgtataacgaactgcagaaagacaagatggccgaggcctacagcgagatcggcatgaagggcgagcggaggcggggcaagggccacgacggcctgtatcagggcctgtccaccgccaccaaggatacctacgacgccctgcacatgcaggccctgcccccaaggctcgagggcggcggagagggcagaggaagtcttctaacatgcggtgacgtggaggagaatcccggccctaggatgcttctcctggtgacaagccttctgctctgtgagttaccacacccagcattcctcctgatcccacgcaaagtgtgtaacggaataggtattggtgaatttaaagactcactctccataaatgctacgaatattaaacacttcaaaaactgcacctccatcagtggcgatctccacatcctgccggtggcatttaggggtgactccttcacacatactcctcctctggatccacaggaactggatattctgaaaaccgtaaaggaaatcacagggtttttgctgattcaggcttggcctgaaaacaggacggacctccatgcctttgagaacctagaaatcatacgcggcaggaccaagcaacatggtcagttttctcttgcagtcgtcagcctgaacataacatccttgggattacgctccctcaaggagataagtgatggagatgtgataatttcaggaaacaaaaatttgtgctatgcaaatacaataaactggaaaaaactgtttgggacctccggtcagaaaaccaaaattataagcaacagaggtgaaaacagctgcaaggccacaggccaggtctgccatgccttgtgctcccccgagggctgctggggcccggagcccagggactgcgtctcttgccggaatgtcagccgaggcagggaatgcgtggacaagtgcaaccttctggagggtgagccaagggagtttgtggagaactctgagtgcatacagtgccacccagagtgcctgcctcaggccatgaacatcacctgcacaggacggggaccagacaactgtatccagtgtgcccactacattgacggcccccactgcgtcaagacctgcccggcaggagtcatgggagaaaacaacaccctggtctggaagtacgcagacgccggccatgtgtgccacctgtgccatccaaactgcacctacggatgcactgggccaggtcttgaaggctgtccaacgaatgggcctaagatcccgtccatcgccactgggatggtgggggccctcctcttgctgctggtggtggccctggggatcggcctcttcatgtga

SEQ ID NO: 11 - protein, 841 aa, synthetic construct
  REGION 1..841: note = Synthetic
MLLLVTSLLLCELPHPAFLLIPDIQMTQTTSSLSASLGDRVTISCRASQDISKYLNWYQQKPDGTVKLLIYHTSRLHSGVPSRFSGSGSGTDYSLTISNLEQEDIATYFCQQGNTLPYTFGGGTKLEITGSTSGSGKPGSGEGSTKGEVKLQESGPGLVAPSQSLSVTCTVSGVSLPDYGVSWIRQPPRKGLEWLGVIWGSETTYYNSALKSRLTIIKDNSKSQVFLKMNSLQTDDTAIYYCAKHYYYGGSYAMDYWGQGTSVTVSSESKYGPPCPPCPMFWVLVVVGGVLACYSLLVTVAFIIFWVKRGRKKLLYIFKQPFMRPVQTTQEEDGCSCRFEEEEGGCELRVKFSRSADAPAYQQGQNQLYNELNLGRREEYDVLDKRRGRDPEMGGKPRRKNPQEGLYNELQKDKMAEAYSEIGMKGERRRGKGHDGLYQGLSTATKDTYDALHMQALPPRLEGGGEGRGSLLTCGDVEENPGPRMLLLVTSLLLCELPHPAFLLIPRKVCNGIGIGEFKDSLSINATNIKHFKNCTSISGDLHILPVAFRGDSFTHTPPLDPQELDILKTVKEITGFLLIQAWPENRTDLHAFENLEIIRGRTKQHGQFSLAVVSLNITSLGLRSLKEISDGDVIISGNKNLCYANTINWKKLFGTSGQKTKIISNRGENSCKATGQVCHALCSPEGCWGPEPRDCVSCRNVSRGRECVDKCNLLEGEPREFVENSECIQCHPECLPQAMNITCTGRGPDNCIQCAHYIDGPHCVKTCPAGVMGENNTLVWKYADAGHVCHLCHPNCTYGCTGPGLEGCPTNGPKIPSIATGMVGALLLLLVVALGIGLFM

SEQ ID NO: 12 - protein, 15 aa, synthetic construct
  REGION 1..15: note = Synthetic
GGGGSGGGGSGGGGS

SEQ ID NO: 13 - protein, 327 aa, Homo sapiens
ASTKGPSVFPLAPCSRSTSESTAALGCLVKDYFPEPVTVSWNSGALTSGVHTFPAVLQSSGLYSLSSVVTVPSSSLGTKTYTCNVDHKPSNTKVDKRVESKYGPPCPSCPAPEFLGGPSVFLFPPKPKDTLMISRTPEVTCVVVDVSQEDPEVQFNWYVDGVEVHNAKTKPREEQFNSTYRVVSVLTVLHQDWLNGKEYKCKVSNKGLPSSIEKTISKAKGQPREPQVYTLPPSQEEMTKNQVSLTCLVKGFYPSDIAVEWESNGQPENNYKTTPPVLDSDGSFFLYSRLTVDKSRWQEGNVFSCSVMHEALHNHYTQKSLSLSLGK

SEQ ID NO: 14 - protein, 220 aa, Homo sapiens
MLRLLLALNLFPSIQVTGNKILVKQSPMLVAYDNAVNLSCKYSYNLFSREFRASLHKGLDSAVEVCVVYGNYSQQLQVYSKTGFNCDGKLGNESVTFYLQNLYVNQTDIYFCKIEVMYPPPYLDNEKSNGTIIHVKGKHLCPSPLFPGPSKPFWVLVVVGGVLACYSLLVTVAFIIFWVRSKRSRLLHSDYMNMTPRRPGPTRKHYQPYAPPRDFAAYRS

SEQ ID NO: 15 - protein, 255 aa, Homo sapiens
MGNSCYNIVATLLLVLNFERTRSLQDPCSNCPAGTFCDNNRNQICSPCPPNSFSSAGGQRTCDICRQCKGVFRTRKECSSTSNAECDCTPGFHCLGAGCSMCEQDCKQGQELTKKGCKDCCFGTFNDQKRGICRPWTNCSLDGKSVLVNGTKERDVVCGPSPADLSPGASSVTPPAPAREPGHSPQIISFFLALTSTALLFLLFFLTLRFSVVKRGRKKLLYIFKQPFMRPVQTTQEEDGCSCRFPEEEEGGCEL

SEQ ID NO: 16 - protein, 164 aa, Homo sapiens
MKWKALFTAAILQAQLPITEAQSFGLLDPKLCYLLDGILFIYGVILTALFLRVKFSRSADAPAYQQGQNQLYNELNLGRREEYDVLDKRRGRDPEMGGKPQRRKNPQEGLYNELQKDKMAEAYSEIGMKGERRRGKGHDGLYQGLSTATKDTYDALHMQALPPR

SEQ ID NO: 17 - protein, 15 aa, Homo sapiens
EPKSCDKTHTCPPCP

SEQ ID NO: 18 - protein, 12 aa, Homo sapiens
ERKCCVECPPCP

SEQ ID NO: 19 - protein, 61 aa, Homo sapiens
ELKTPLGDTHTCPRCPEPKSCDTPPPCPRCPEPKSCDTPPPCPRCPEPKSCDTPPPCPRCP

SEQ ID NO: 20 - protein, 12 aa, Homo sapiens
ESKYGPPCPSCP

SEQ ID NO: 21 - protein, 12 aa, synthetic construct
  REGION 1..12: note = Synthetic
ESKYGPPCPPCP

SEQ ID NO: 22 - DNA, 26 bp, synthetic construct
  misc_feature 1..26: note = Primer
  source 1..26: mol_type = other DNA
atcaaaagaatagaccgagatagggt

SEQ ID NO: 23 - DNA, 26 bp, synthetic construct
  misc_feature 1..26: note = Primer
  source 1..26: mol_type = other DNA
ccgtacctttaagaccaatgacttac

SEQ ID NO: 24 - DNA, 18 bp, synthetic construct
  misc_feature 1..18: note = Primer
  source 1..18: mol_type = other DNA
ttgagagttttcgccccg

SEQ ID NO: 25 - DNA, 24 bp, synthetic construct
  misc_feature 1..24: note = Primer
  source 1..24: mol_type = other DNA
aatagacagatcgctgagataggt

SEQ ID NO: 26 - DNA, 18 bp, synthetic construct
  misc_feature 1..18: note = Primer
  source 1..18: mol_type = other DNA
caggtatccggtaagcgg

SEQ ID NO: 27 - DNA, 19 bp, synthetic construct
  misc_feature 1..19: note = Primer
  source 1..19: mol_type = other DNA
cgaccagcaaccatagtcc

SEQ ID NO: 28 - DNA, 18 bp, synthetic construct
  misc_feature 1..18: note = Primer
  source 1..18: mol_type = other DNA
tagcggtttgactcacgg

SEQ ID NO: 29 - DNA, 20 bp, synthetic construct
  misc_feature 1..20: note = Primer
  source 1..20: mol_type = other DNA
gcagggagctagaacgattc

SEQ ID NO: 30 - DNA, 22 bp, synthetic construct
  misc_feature 1..22: note = Primer
  source 1..22: mol_type = other DNA
attgtctggtatagtgcagcag

SEQ ID NO: 31 - DNA, 16 bp, synthetic construct
  misc_feature 1..16: note = Primer
  source 1..16: mol_type = other DNA
tcgcaacgggtttgcc

SEQ ID NO: 32 - DNA, 21 bp, synthetic construct
  misc_feature 1..21: note = Primer
  source 1..21: mol_type = other DNA
aggaagatatcgccacctact

SEQ ID NO: 33 - DNA, 20 bp, synthetic construct
  misc_feature 1..20: note = Primer
  source 1..20: mol_type = other DNA
cgggtgaagttcagcagaag

SEQ ID NO: 34 - DNA, 20 bp, synthetic construct
  misc_feature 1..20: note = Primer
  source 1..20: mol_type = other DNA
actgtgtttgctgacgcaac

SEQ ID NO: 35 - DNA, 20 bp, synthetic construct
  misc_feature 1..20: note = Primer
  source 1..20: mol_type = other DNA
atgcttctcctggtgacaag

SEQ ID NO: 36 - protein, 18 aa, synthetic construct
  REGION 1..18: note = Synthetic
GSTSGSGKPGSGEGSTKG

SEQ ID NO: 37 - DNA, 10051 bp, synthetic construct
  misc_feature 1..10051: note = Synthetic
  source 1..10051: mol_type = other DNA
gttagaccagatctgagcctgggagctctctggctaactagggaacccactgcttaagcctcaataaagcttgccttgagtgcttcaagtagtgtgtgcccgtctgttgtgtgactctggtaactagagatccctcagacccttttagtcagtgtggaaaatctctagcagtggcgcccgaacagggacttgaaagcgaaagggaaaccagaggagctctctcgacgcaggactcggcttgctgaagcgcgcacggcaagaggcgaggggcggcgactggtgagtacgccaaaaattttgactagcggaggctagaaggagagagatgggtgcgagagcgtcagtattaagcgggggagaattagatcgatgggaaaaaattcggttaaggccagggggaaagaaaaaatataaattaaaacatatagtatgggcaagcagggagctagaacgattcgcagttaatcctggcctgttagaaacatcagaaggctgtagacaaatactgggacagctacaaccatcccttcagacaggatcagaagaacttagatcattatataatacagtagcaaccctctattgtgtgcatcaaaggatagagataaaagacaccaaggaagctttagacaagatagaggaagagcaaaacaaaagtaagaaaaaagcacagcaagcagcagctgacacaggacacagcaatcaggtcagccaaaattaccctatagtgcagaacatccaggggcaaatggtacatcaggccatatcacctagaactttaaatgcatgggtaaaagtagtagaagagaaggctttcagcccagaagtgatacccatgttttcagcattatcagaaggagccaccccacaagatttaaacaccatgctaaacacagtggggggacatcaagcagccatgcaaatgttaaaagagaccatcaatgaggaagctgcaggcaaagagaagagtggtgcagagagaaaaaagagcagtgggaataggagctttgttccttgggttcttgggagcagcaggaagcactatgggcgcagcgtcaatgacgctgacggtacaggccagacaattattgtctggtatagtgcagcagcagaacaatttgctgagggctattgaggcgcaacagcatctgttgcaactcacagtctggggcatcaagcagctccaggcaagaatcctggctgtggaaagatacctaaaggatcaacagctcctggggatttggggttgctctggaaaactcatttgcaccactgctgtgccttggatctacaaatggcagtattcatccacaattttaaaagaaaaggggggattggggggtacagtgcaggggaaagaatagtagacataatagcaacagacatacaaactaaagaattacaaaaacaaattacaaaaattcaaaattttcgggtttattacagggacagcagagatccagtttggggatcaattgcatgaagaatctgcttagggttaggcgttttgcgctgcttcgcgaggatctgcgatcgctccggtgcccgtcagtgggcagagcgcacatcgcccacagtccccgagaagttggggggaggggtcggcaattgaaccggtgcctagagaaggtggcgcggggtaaactgggaaagtgatgtcgtgtactggctccgcctttttcccgagggtgggggagaaccgtatataagtgcagtagtcgccgtgaacgttctttttcgcaacgggtttgccgccagaacacagctgaagcttcgaggggctcgcatctctccttcacgcgcccgccgccctacctgaggccgccatccacgccggttgagtcgcgttctgccgcctcccgcctgtggtgcctcctgaactgcgtccgccgtctaggtaagtttaaagctcaggtcgagaccgggcctttgtccggcgctcccttggagcctacctagactcagccggctctccacgctttgcctgaccctgcttgctcaactctacgtctttgtttcgttttctgttctgcgccgttacagatccaagctgtgaccggcgcctacggctagcgaattcctcgaggccaccatgctgctgctggtgacaagcctgctgctgtgcgagctgccccaccccgcctttctgctgatcccccaggaacagctcgtcgaaagcggcggcagactggtgacacctggcggcagcctgaccctgagctgcaaggccagcggcttcgacttcagcgcctactacatgagctgggtccgccaggcccctggcaagggactggaatggatcgccaccatctaccccagcagcggcaagacctactacgccacctgggtgaacggacggttcaccatctccagcgacaacgcccagaacaccgtggacctgcagatgaacagcctgacagccgccgaccgggccacctacttttgcgccagagacagctacgccgacgacggcgccctgttcaacatctggggccctggcaccctggtgacaatctctagcggcggaggcggatctggtggcggaggaagtggcggcggaggatctgagctggtgctgacccagagcccctctgtgtctgctgccctgggaagccctgccaagatcacctgtaccctgagcagcgcccacaagaccgacaccatcgactggtatcagcagctgcagggcgaggcccccagatacctgatgcaggtgcagagcgacggcagctacaccaagaggccaggcgtgcccgaccggttcagcggatctagctctggcgccgaccgctacctgatcatccccagcgtgcaggccgatgacgaggccgattactactgtggcgccgactacatcggcggctacgtgttcggcggaggcacccagctgaccgtgaccggcgagtctaagtacggaccgccctgccccccttgccctgcccccgagttcctgggcggacccagcgtgttcctgttcccccccaagcccaaggacaccctgatgatcagccggacccccgaggtgacctgcgtggtggtggacgtgagccaggaagatcccgaggtccagttcaattggtacgtggacggcgtggaagtgcacaacgccaagaccaagcccagagaggaacagttcaacagcacctaccgggtggtgtctgtgctgaccgtgctgcaccaggactggctgaacggcaaagaatacaagtgcaaggtgtccaacaagggcctgcccagcagcatcgaaaagaccatcagcaaggccaagggccagcctcgcgagccccaggtgtacaccctgcctccctcccaggaagagatgaccaagaaccaggtgtccctgacctgcctggtgaagggcttctaccccagcgacatcgccgtggagtgggagagcaacggccagcctgagaacaactacaagaccacccctcccgtgctggacagcgacggcagcttcttcctgtacagccggctgaccgtggacaagagccggtggcaggaaggcaacgtctttagctgcagcgtgatgcacgaggccctgcacaaccactacacccagaagagcctgagcctgtccctgggcaagatgttctgggtgctggtggtggtgggcggggtgctggcctgctacagcctgctggtgacagtggccttcatcatcttttgggtgaaacggggcagaaagaaactcctgtatatattcaaacaaccatttatgagaccagtacaaactactcaagaggaagatggctgtagctgccgatttccagaagaagaagaaggaggatgtgaactgcgggtgaagttcagcagaagcgccgacgcccctgcctaccagcagggccagaatcagctgtacaacgagctgaacctgggcagaagggaagagtacgacgtcctggataagcggagaggccgggaccctgagatgggcggcaagcctcggcggaagaacccccaggaaggcctgtataacgaactgcagaaagacaagatggccgaggcctacagcgagatcggcatgaagggcgagcggaggcggggcaagggccacgacggcctgtatcagggcctgtccaccgccaccaaggatacctacgacgccctgcacatgcaggccctgcccccaaggctcgagggcggcggagagggcagaggaagtcttctaacatgcggtgacgtggaggagaatcccggccctaggatgcttctcctggtgacaagccttctgctctgtgagttaccacacccagcattcctcctgatcccacgcaaagtgtgtaacggaataggtattggtgaatttaaagactcactctccataaatgctacgaatattaaacacttcaaaaactgcacctccatcagtggcgatctccacatcctgccggtggcatttaggggtgactccttcacacatactcctcctctggatccacaggaactggatattctgaaaaccgtaaaggaaatcacagggtttttgctgattcaggcttggcctgaaaacaggacggacctccatgcctttgagaacctagaaatcatacgcggcaggaccaagcaacatggtcagttttctcttgcagtcgtcagcctgaacataacatccttgggattacgctccctcaaggagataagtgatggagatgtgataatttcaggaaacaaaaatttgtgctatgcaaatacaataaactggaaaaaactgtttgggacctccggtcagaaaaccaaaattataagcaacagaggtgaaaacagctgcaaggccacaggccaggtctgccatgccttgtgctcccccgagggctgctggggcccggagcccagggactgcgtctcttgccggaatgtcagccgaggcagggaatgcgtggacaagtgcaaccttctggagggtgagccaagggagtttgtggagaactctgagtgcatacagtgccacccagagtgcctgcctcaggccatgaacatcacctgcacaggacggggaccagacaactgtatccagtgtgcccactacattgacggcccccactgcgtcaagacctgcccggcaggagtcatgggagaaaacaacaccctggtctggaagtacgcagacgccggccatgtgtgccacctgtgccatccaaactgcacctacggatgcactgggccaggtcttgaaggctgtccaacgaatgggcctaagatcccgtccatcgccactgggatggtgggggccctcctcttgctgctggtggtggccctggggatcggcctcttcatgtgagcggccgctctagacccgggctgcaggaattcgatatcaagcttatcgataatcaacctctggattacaaaatttgtgaaagattgactggtattcttaactatgttgctccttttacgctatgtggatacgctgctttaatgcctttgtatcatgctattgcttcccgtatggctttcattttctcctccttgtataaatcctggttgctgtctctttatgaggagttgtggcccgttgtcaggcaacgtggcgtggtgtgcactgtgtttgctgacgcaacccccactggttggggcattgccaccacctgtcagctcctttccgggactttcgctttccccctccctattgccacggcggaactcatcgccgcctgccttgcccgctgctggacaggggctcggctgttgggcactgacaattccgtggtgttgtcggggaaatcatcgtcctttccttggctgctcgcctgtgttgccacctggattctgcgcgggacgtccttctgctacgtcccttcggccctcaatccagcggaccttccttcccgcggcctgctgccggctctgcggcctcttccgcgtcttcgccttcgccctcagacgagtcggatctccctttgggccgcctccccgcatcgataccgtcgactagccgtacctttaagaccaatgacttacaaggcagctgtagatcttagccactttttaaaagaaaaggggggactggaagggctaattcactcccaaagaagacaagatctgctttttgcctgtactgggtctctctggttagaccagatctgagcctgggagctctctggctaactagggaacccactgcttaagcctcaataaagcttgccttgagtgcttcaagtagtgtgtgcccgtctgttgtgtgactctggtaactagagatccctcagacccttttagtcagtgtggaaaatctctagcagaattcgatatcaagcttatcgataccgtcgacctcgagggggggcccggtacccaattcgccctatagtgagtcgtattacaattcactggccgtcgttttacaacgtcgtgactgggaaaaccctggcgttacccaacttaatcgccttgcagcacatccccctttcgccagctggcgtaatagcgaagaggcccgcaccgatcgcccttcccaacagttgcgcagcctgaatggcgaatggaaattgtaagcgttaatattttgttaaaattcgcgttaaatttttgttaaatcagctcattttttaaccaataggccgaaatcggcaaaatcccttataaatcaaaagaatagaccgagatagggttgagtgttgttccagtttggaacaagagtccactattaaagaacgtggactccaacgtcaaagggcgaaaaaccgtctatcagggcgatggcccactacgtgaaccatcaccctaatcaagttttttggggtcgaggtgccgtaaagcactaaatcggaaccctaaagggagcccccgatttagagcttgacggggaaagccggcgaacgtggcgagaaaggaagggaagaaagcgaaaggagcgggcgctagggcgctggcaagtgtagcggtcacgctgcgcgtaaccaccacacccgccgcgcttaatgcgccgctacagggcgcgtcaggtggcacttttcggggaaatgtgcgcggaacccctatttgtttatttttctaaatacattcaaatatgtatccgctcatgagacaataaccctgataaatgcttcaataatattgaaaaaggaagagtatgagtattcaacatttccgtgtcgcccttattcccttttttgcggcattttgccttcctgtttttgctcacccagaaacgctggtgaaagtaaaagatgctgaagatcagttgggtgcacgagtgggttacatcgaactggatctcaacagcggtaagatccttgagagttttcgccccgaagaacgttttccaatgatgagcacttttaaagttctgctatgtggcgcggtattatcccgtattgacgccgggcaagagcaactcggtcgccgcatacactattctcagaatgacttggttgagtactcaccagtcacagaaaagcatcttacggatggcatgacagtaagagaattatgcagtgctgccataaccatgagtgataacactgcggccaacttacttctgacaacgatcggaggaccgaaggagctaaccgcttttttgcacaacatgggggatcatgtaactcgccttgatcgttgggaaccggagctgaatgaagccataccaaacgacgagcgtgacaccacgatgcctgtagcaatggcaacaacgttgcgcaaactattaactggcgaactacttactctagcttcccggcaacaattaatagactggatggaggcggataaagttgcaggaccacttctgcgctcggcccttccggctggctggtttattgctgataaatctggagccggtgagcgtgggtctcgcggtatcattgcagcactggggccagatggtaagccctcccgtatcgtagttatctacacgacggggagtcaggcaactatggatgaacgaaatagacagatcgctgagataggtgcctcactgattaagcattggtaactgtcagaccaagtttactcatatatactttagattgatttaaaacttcatttttaatttaaaaggatctaggtgaagatcctttttgataatctcatgaccaaaatcccttaacgtgagttttcgttccactgagcgtcagaccccgtagaaaagatcaaaggatcttcttgagatcctttttttctgcgcgtaatctgctgcttgcaaacaaaaaaaccaccgctaccagcggtggtttgtttgccggatcaagagctaccaactctttttccgaaggtaactggcttcagcagagcgcagataccaaatactgttcttctagtgtagccgtagttaggccaccacttcaagaactctgtagcaccgcctacatacctcgctctgctaatcctgttaccagtggctgctgccagtggcgataagtcgtgtcttaccgggttggactcaagacgatagttaccggataaggcgcagcggtcgggctgaacggggggttcgtgcacacagcccagcttggagcgaacgacctacaccgaactgagatacctacagcgtgagctatgagaaagcgccacgcttcccgaagggagaaaggcggacaggtatccggtaagcggcagggtcggaacaggagagcgcacgagggagcttccagggggaaacgcctggtatctttatagtcctgtcgggtttcgccacctctgacttgagcgtcgatttttgtgatgctcgtcaggggggcggagcctatggaaaaacgccagcaacgcggcctttttacggttcctggccttttgctggccttttgctcacatgttctttcctgcgttatcccctgattctgtggataaccgtattaccgcctttgagtgagctgataccgctcgccgcagccgaacgaccgagcgcagcgagtcagtgagcgaggaagcggaagagcgcccaatacgcaaaccgcctctccccgcgcgttggccgattcattaatgcagctggcacgacaggtttcccgactggaaagcgggcagtgagcgcaacgcaattaatgtgagttagctcactcattaggcaccccaggctttacactttatgcttccggctcgtatgttgtgtggaattgtgagcggataacaatttcacacaggaaacagctatgaccatgattacgccaagctcgaaattaaccctcactaaagggaacaaaagctggagctccaccgcggtggcggcctcgaggtcgagatccggtcgaccagcaaccatagtcccgcccctaactccgcccatcccgcccctaactccgcccagttccgcccattctccgccccatggctgactaattttttttatttatgcagaggccgaggccgcctcggcctctgagctattccagaagtagtgaggaggcttttttggaggcctaggcttttgcaaaaagcttcgacggtatcgattggctcatgtccaacattaccgccatgttgacattgattattgactagttattaatagtaatcaattacggggtcattagttcatagcccatatatggagttccgcgttacataacttacggtaaatggcccgcctggctgaccgcccaacgacccccgcccattgacgtcaataatgacgtatgttcccatagtaacgccaatagggactttccattgacgtcaatgggtggagtatttacggtaaactgcccacttggcagtacatcaagtgtatcatatgccaagtacgccccctattgacgtcaatgacggtaaatggcccgcctggcattatgcccagtacatgaccttatgggactttcctacttggcagtacatctacgtattagtcatcgctattaccatggtgatgcggttttggcagtacatcaatgggcgtggatagcggtttgactcacggggatttccaagtctccaccccattgacgtcaatgggagtttgttttggcaccaaaatcaacgggactttccaaaatgtcgtaacaactccgccccattgacgcaaatgggcggtaggcgtgtacggaattcggagtggcgagccctcagatcctgcatataagcagctgctttttgcctgtactgggtctctctg

SEQ ID NO: 38 - protein, 1062 aa, synthetic construct
  REGION 1..1062: note = Synthetic
MLLLVTSLLLCELPHPAFLLIPQEQLVESGGRLVTPGGSLTLSCKASGFDFSAYYMSWVRQAPGKGLEWIATIYPSSGKTYYATWVNGRFTISSDNAQNTVDLQMNSLTAADRATYFCARDSYADDGALFNIWGPGTLVTISSGGGGSGGGGSGGGGSELVLTQSPSVSAALGSPAKITCTLSSAHKTDTIDWYQQLQGEAPRYLMQVQSDGSYTKRPGVPDRFSGSSSGADRYLIIPSVQADDEADYYCGADYIGGYVFGGGTQLTVTGESKYGPPCPPCPAPEFLGGPSVFLFPPKPKDTLMISRTPEVTCVVVDVSQEDPEVQFNWYVDGVEVHNAKTKPREEQFNSTYRVVSVLTVLHQDWLNGKEYKCKVSNKGLPSSIEKTISKAKGQPREPQVYTLPPSQEEMTKNQVSLTCLVKGFYPSDIAVEWESNGQPENNYKTTPPVLDSDGSFFLYSRLTVDKSRWQEGNVFSCSVMHEALHNHYTQKSLSLSLGKMFWVLVVVGGVLACYSLLVTVAFIIFWVKRGRKKLLYIFKQPFMRPVQTTQEEDGCSCRFPEEEEGGCELRVKFSRSADAPAYQQGQNQLYNELNLGRREEYDVLDKRRGRDPEMGGKPRRKNPQEGLYNELQKDKMAEAYSEIGMKGERRRGKGHDGLYQGLSTATKDTYDALHMQALPPRLEGGGEGRGSLLTCGDVEENPGPRMLLLVTSLLLCELPHPAFLLIPRKVCNGIGIGEFKDSLSINATNIKHFKNCTSISGDLHILPVAFRGDSFTHTPPLDPQELDILKTVKEITGFLLIQAWPENRTDLHAFENLEIIRGRTKQHGQFSLAVVSLNITSLGLRSLKEISDGDVIISGNKNLCYANTINWKKLFGTSGQKTKIISNRGENSCKATGQVCHALCSPEGCWGPEPRDCVSCRNVSRGRECVDKCNLLEGEPREFVENSECIQCHPECLPQAMNITCTGRGPDNCIQCAHYIDGPHCVKTCPAGVMGENNTLVWKYADAGHVCHLCHPNCTYGCTGPGLEGCPTNGPKIPSIATGMVGALLLLLVVALGIGLFM

SEQ ID NO: 39 - DNA, 9721 bp, synthetic construct
  misc_feature 1..9721: note = Synthetic
  source 1..9721: mol_type = other DNA
gttagaccagatctgagcctgggagctctctggctaactagggaacccactgcttaagcctcaataaagcttgccttgagtgcttcaagtagtgtgtgcccgtctgttgtgtgactctggtaactagagatccctcagacccttttagtcagtgtggaaaatctctagcagtggcgcccgaacagggacttgaaagcgaaagggaaaccagaggagctctctcgacgcaggactcggcttgctgaagcgcgcacggcaagaggcgaggggcggcgactggtgagtacgccaaaaattttgactagcggaggctagaaggagagagatgggtgcgagagcgtcagtattaagcgggggagaattagatcgatgggaaaaaattcggttaaggccagggggaaagaaaaaatataaattaaaacatatagtatgggcaagcagggagctagaacgattcgcagttaatcctggcctgttagaaacatcagaaggctgtagacaaatactgggacagctacaaccatcccttcagacaggatcagaagaacttagatcattatataatacagtagcaaccctctattgtgtgcatcaaaggatagagataaaagacaccaaggaagctttagacaagatagaggaagagcaaaacaaaagtaagaaaaaagcacagcaagcagcagctgacacaggacacagcaatcaggtcagccaaaattaccctatagtgcagaacatccaggggcaaatggtacatcaggccatatcacctagaactttaaatgcatgggtaaaagtagtagaagagaaggctttcagcccagaagtgatacccatgttttcagcattatcagaaggagccaccccacaagatttaaacaccatgctaaacacagtggggggacatcaagcagccatgcaaatgttaaaagagaccatcaatgaggaagctgcaggcaaagagaagagtggtgcagagagaaaaaagagcagtgggaataggagctttgttccttgggttcttgggagcagcaggaagcactatgggcgcagcgtcaatgacgctgacggtacaggccagacaattattgtctggtatagtgcagcagcagaacaatttgctgagggctattgaggcgcaacagcatctgttgcaactcacagtctggggcatcaagcagctccaggcaagaatcctggctgtggaaagatacctaaaggatcaacagctcctggggatttggggttgctctggaaaactcatttgcaccactgctgtgccttggatctacaaatggcagtattcatccacaattttaaaagaaaaggggggattggggggtacagtgcaggggaaagaatagtagacataatagcaacagacatacaaactaaagaattacaaaaacaaattacaaaaattcaaaattttcgggtttattacagggacagcagagatccagtttggggatcaattgcatgaagaatctgcttagggttaggcgttttgcgctgcttcgcgaggatctgcgatcgctccggtgcccgtcagtgggcagagcgcacatcgcccacagtccccgagaagttggggggaggggtcggcaattgaaccggtgcctagagaaggtggcgcggggtaaactgggaaagtgatgtcgtgtactggctccgcctttttcccgagggtgggggagaaccgtatataagtgcagtagtcgccgtgaacgttctttttcgcaacgggtttgccgccagaacacagctgaagcttcgaggggctcgcatctctccttcacgcgcccgccgccctacctgaggccgccatccacgccggttgagtcgcgttctgccgcctcccgcctgtggtgcctcctgaactgcgtccgccgtctaggtaagtttaaagctcaggtcgagaccgggcctttgtccggcgctcccttggagcctacctagactcagccggctctccacgctttgcctgaccctgcttgctcaactctacgtctttgtttcgttttctgttctgcgccgttacagatccaagctgtgaccggcgcctacggctagcgaattcctcgaggccaccatgctgctgctggtgacaagcctgctgctgtgcgagctgccccaccccgcctttctgctgatcccccaggaacagctcgtcgaaagcggcggcagactggtgacacctggcggcagcctgaccctgagctgcaaggccagcggcttcgacttcagcgcctactacatgagctgggtccgccaggcccctggcaagggactggaatggatcgccaccatctaccccagcagcggcaagacctactacgccacctgggtgaacggacggttcaccatctccagcgacaacgcccagaacaccgtggacctgcagatgaacagcctgacagccgccgaccgggccacctacttttgcgccagagacagctacgccgacgacggcgccctgttcaacatctggggccctggcaccctggtgacaatctctagcggcggaggcggatctggtggcggaggaagtggcggcggaggatctgagctggtgctgacccagagcccctctgtgtctgctgccctgggaagccctgccaagatcacctgtaccctgagcagcgcccacaagaccgacaccatcgactggtatcagcagctgcagggcgaggcccccagatacctgatgcaggtgcagagcgacggcagctacaccaagaggccaggcgtgcccgaccggttcagcggatctagctctggcgccgaccgctacctgatcatccccagcgtgcaggccgatgacgaggccgattactactgtggcgccgactacatcggcggctacgtgttcggcggaggcacccagctgaccgtgaccggcgagtctaagtacggaccgccctgccccccttgccctggccagcctcgcgagccccaggtgtacaccctgcctccctcccaggaagagatgaccaagaaccaggtgtccctgacctgcctggtgaagggcttctaccccagcgacatcgccgtggagtgggagagcaacggccagcctgagaacaactacaagaccacccctcccgtgctggacagcgacggcagcttcttcctgtacagccggctgaccgtggacaagagccggtggcaggaaggcaacgtctttagctgcagcgtgatgcacgaggccctgcacaaccactacacccagaagagcctgagcctgtccctgggcaagatgttctgggtgctggtggtggtgggcggggtgctggcctgctacagcctgctggtgacagtggccttcatcatcttttgggtgaaacggggcagaaagaaactcctgtatatattcaaacaaccatttatgagaccagtacaaactactcaagaggaagatggctgtagctgccgatttccagaagaagaagaaggaggatgtgaactgcgggtgaagttcagcagaagcgccgacgcccctgcctaccagcagggccagaatcagctgtacaacgagctgaacctgggcagaagggaagagtacgacgtcctggataagcggagaggccgggaccctgagatgggcggcaagcctcggcggaagaacccccaggaaggcctgtataacgaactgcagaaagacaagatggccgaggcctacagcgagatcggcatgaagggcgagcggaggcggggcaagggccacgacggcctgtatcagggcctgtccaccgccaccaaggatacctacgacgccctgcacatgcaggccctgcccccaaggctcgagggcggcggagagggcagaggaagtcttctaacatgcggtgacgtggaggagaatcccggccctaggatgcttctcctggtgacaagccttctgctctgtgagttaccacacccagcattcctcctgatcccacgcaaagtgtgtaacggaataggtattggtgaatttaaagactcactctccataaatgctacgaatattaaacacttcaaaaactgcacctccatcagtggcgatctccacatcctgccggtggcatttaggggtgactccttcacacatactcctcctctggatccacaggaactggatattctgaaaaccgtaaaggaaatcacagggtttttgctgattcaggcttggcctgaaaacaggacggacctccatgcctttgagaacctagaaatcatacgcggcaggaccaagcaacatggtcagttttctcttgcagtcgtcagcctgaacataacatccttgggattacgctccctcaaggagataagtgatggagatgtgataatttcaggaaacaaaaatttgtgctatgcaaatacaataaactggaaaaaactgtttgggacctccggtcagaaaaccaaaattataagcaacagaggtgaaaacagctgcaaggccacaggccaggtctgccatgccttgtgctcccccgagggctgctggggcccggagcccagggactgcgtctcttgccggaatgtcagccgaggcagggaatgcgtggacaagtgcaaccttctggagggtgagccaagggagtttgtggagaactctgagtgcatacagtgccacccagagtgcctgcctcaggccatgaacatcacctgcacaggacggggaccagacaactgtatccagtgtgcccactacattgacggcccccactgcgtcaagacctgcccggcaggagtcatgggagaaaacaacaccctggtctggaagtacgcagacgccggccatgtgtgccacctgtgccatccaaactgcacctacggatgcactgggccaggtcttgaaggctgtccaacgaatgggcctaagatcccgtccatcgccactgggatggtgggggccctcctcttgctgctggtggtggccctggggatcggcctcttcatgtgagcggccgctctagacccgggctgcaggaattcgatatcaagcttatcgataatcaacctctggattacaaaatttgtgaaagattgactggtattcttaactatgttgctccttttacgctatgtggatacgctgctttaatgcctttgtatcatgctattgcttcccgtatggctttcattttctcctccttgtataaatcctggttgctgtctctttatgaggagttgtggcccgttgtcaggcaacgtggcgtggtgtgcactgtgtttgctgacgcaacccccactggttggggcattgccaccacctgtcagctcctttccgggactttcgctttccccctccctattgccacggcggaactcatcgccgcctgccttgcccgctgctggacaggggctcggctgttgggcactgacaattccgtggtgttgtcggggaaatcatcgtcctttccttggctgctcgcctgtgttgccacctggattctgcgcgggacgtccttctgctacgtcccttcggccctcaatccagcggaccttccttcccgcggcctgctgccggctctgcggcctcttccgcgtcttcgccttcgccctcagacgagtcggatctccctttgggccgcctccccgcatcgataccgtcgactagccgtacctttaagaccaatgacttacaaggcagctgtagatcttagccactttttaaaagaaaaggggggactggaagggctaattcactcccaaagaagacaagatctgctttttgcctgtactgggtctctctggttagaccagatctgagcctgggagctctctggctaactagggaacccactgcttaagcctcaataaagcttgccttgagtgcttcaagtagtgtgtgcccgtctgttgtgtgactctggtaactagagatccctcagacccttttagtcagtgtggaaaatctctagcagaattcgatatcaagcttatcgataccgtcgacctcgagggggggcccggtacccaattcgccctatagtgagtcgtattacaattcactggccgtcgttttacaacgtcgtgactgggaaaaccctggcgttacccaacttaatcgccttgcagcacatccccctttcgccagctggcgtaatagcgaagaggcccgcaccgatcgcccttcccaacagttgcgcagcctgaatggcgaatggaaattgtaagcgttaatattttgttaaaattcgcgttaaatttttgttaaatcagctcattttttaaccaataggccgaaatcggcaaaatcccttataaatcaaaagaatagaccgagatagggttgagtgttgttccagtttggaacaagagtccactattaaagaacgtggactccaacgtcaaagggcgaaaaaccgtctatcagggcgatggcccactacgtgaaccatcaccctaatcaagttttttggggtcgaggtgccgtaaagcactaaatcggaaccctaaagggagcccccgatttagagcttgacggggaaagccggcgaacgtggcgagaaaggaagggaagaaagcgaaaggagcgggcgctagggcgctggcaagtgtagcggtcacgctgcgcgtaaccaccacacccgccgcgcttaatgcgccgctacagggcgcgtcaggtggcacttttcggggaaatgtgcgcggaacccctatttgtttatttttctaaatacattcaaatatgtatccgctcatgagacaataaccctgataaatgcttcaataatattgaaaaaggaagagtatgagtattcaacatttccgtgtcgcccttattcccttttttgcggcattttgccttcctgtttttgctcacccagaaacgctggtgaaagtaaaagatgctgaagatcagttgggtgcacgagtgggttacatcgaactggatctcaacagcggtaagatccttgagagttttcgccccgaagaacgttttccaatgatgagcacttttaaagttctgctatgtggcgcggtattatcccgtattgacgccgggcaagagcaactcggtcgccgcatacactattctcagaatgacttggttgagtactcaccagtcacagaaaagcatcttacggatggcatgacagtaagagaattatgcagtgctgccataaccatgagtgataacactgcggccaacttacttctgacaacgatcggaggaccgaaggagctaaccgcttttttgcacaacatgggggatcatgtaactcgccttgatcgttgggaaccggagctgaatgaagccataccaaacgacgagcgtgacaccacgatgcctgtagcaatggcaacaacgttgcgcaaactattaactggcgaactacttactctagcttcccggcaacaattaatagactggatggaggcggataaagttgcaggaccacttctgcgctcggcccttccggctggctggtttattgctgataaatctggagccggtgagcgtgggtctcgcggtatcattgcagcactggggccagatggtaagccctcccgtatcgtagttatctacacgacggggagtcaggcaactatggatgaacgaaatagacagatcgctgagataggtgcctcactgattaagcattggtaactgtcagaccaagtttactcatatatactttagattgatttaaaacttcatttttaatttaaaaggatctaggtgaagatcctttttgataatctcatgaccaaaatcccttaacgtgagttttcgttccactgagcgtcagaccccgtagaaaagatcaaaggatcttcttgagatcctttttttctgcgcgtaatctgctgcttgcaaacaaaaaaaccaccgctaccagcggtggtttgtttgccggatcaagagctaccaactctttttccgaaggtaactggcttcagcagagcgcagataccaaatactgttcttctagtgtagccgtagttaggccaccacttcaagaactctgtagcaccgcctacatacctcgctctgctaatcctgttaccagtggctgctgccagtggcgataagtcgtgtcttaccgggttggactcaagacgatagttaccggataaggcgcagcggtcgggctgaacggggggttcgtgcacacagcccagcttggagcgaacgacctacaccgaactgagatacctacagcgtgagctatgagaaagcgccacgcttcccgaagggagaaaggcggacaggtatccggtaagcggcagggtcggaacaggagagcgcacgagggagcttccagggggaaacgcctggtatctttatagtcctgtcgggtttcgccacctctgacttgagcgtcgatttttgtgatgctcgtcaggggggcggagcctatggaaaaacgccagcaacgcggcctttttacggttcctggccttttgctggccttttgctcacatgttctttcctgcgttatcccctgattctgtggataaccgtattaccgcctttgagtgagctgataccgctcgccgcagccgaacgaccgagcgcagcgagtcagtgagcgaggaagcggaagagcgcccaatacgcaaaccgcctctccccgcgcgttggccgattcattaatgcagctggcacgacaggtttcccgactggaaagcgggcagtgagcgcaacgcaattaatgtgagttagctcactcattaggcaccccaggctttacactttatgcttccggctcgtatgttgtgtggaattgtgagcggataacaatttcacacaggaaacagctatgaccatgattacgccaagctcgaaattaaccctcactaaagggaacaaaagctggagctccaccgcggtggcggcctcgaggtcgagatccggtcgaccagcaaccatagtcccgcccctaactccgcccatcccgcccctaactccgcccagttccgcccattctccgccccatggctgactaattttttttatttatgcagaggccgaggccgcctcggcctctgagctattccagaagtagtgaggaggcttttttggaggcctaggcttttgcaaaaagcttcgacggtatcgattggctcatgtccaacattaccgccatgttgacattgattattgactagttattaatagtaatcaattacggggtcattagttcatagcccatatatggagttccgcgttacataacttacggtaaatggcccgcctggctgaccgcccaacgacccccgcccattgacgtcaataatgacgtatgttcccatagtaacgccaatagggactttccattgacgtcaatgggtggagtatttacggtaaactgcccacttggcagtacatcaagtgtatcatatgccaagtacgccccctattgacgtcaatgacggtaaatggcccgcctggcattatgcccagtacatgaccttatgggactttcctacttggcagtacatctacgtattagtcatcgctattaccatggtgatgcggttttggcagtacatcaatgggcgtggatagcggtttgactcacggggatttccaagtctccaccccattgacgtcaatgggagtttgttttggcaccaaaatcaacgggactttccaaaatgtcgtaacaactccgccccattgacgcaaatgggcggtaggcgtgtacggaattcggagtggcgagccctcagatcctgcatataagcagctgctttttgcctgtactgggtctctctg

SEQ ID NO: 40 - protein, 952 aa, synthetic construct
  REGION 1..952: note = Synthetic
MLLLVTSLLLCELPHPAFLLIPQEQLVESGGRLVTPGGSLTLSCKASGFDFSAYYMSWVRQAPGKGLEWIATIYPSSGKTYYATWVNGRFTISSDNAQNTVDLQMNSLTAADRATYFCARDSYADDGALFNIWGPGTLVTISSGGGGSGGGGSGGGGSELVLTQSPSVSAALGSPAKITCTLSSAHKTDTIDWYQQLQGEAPRYLMQVQSDGSYTKRPGVPDRFSGSSSGADRYLIIPSVQADDEADYYCGADYIGGYVFGGGTQLTVTGESKYGPPCPPCPGQPREPQVYTLPPSQEEMTKNQVSLTCLVKGFYPSDIAVEWESNGQPENNYKTTPPVLDSDGSFFLYSRLTVDKSRWQEGNVFSCSVMHEALHNHYTQKSLSLSLGKMFWVLVVVGGVLACYSLLVTVAFIIFWVKRGRKKLLYIFKQPFMRPVQTTQEEDGCSCRFPEEEEGGCELRVKFSRSADAPAYQQGQNQLYNELNLGRREEYDVLDKRRGRDPEMGGKPRRKNPQEGLYNELQKDKMAEAYSEIGMKGERRRGKGHDGLYQGLSTATKDTYDALHMQALPPRLEGGGEGRGSLLTCGDVEENPGPRMLLLVTSLLLCELPHPAFLLIPRKVCNGIGIGEFKDSLSINATNIKHFKNCTSISGDLHILPVAFRGDSFTHTPPLDPQELDILKTVKEITGFLLIQAWPENRTDLHAFENLEIIRGRTKQHGQFSLAVVSLNITSLGLRSLKEISDGDVIISGNKNLCYANTINWKKLFGTSGQKTKIISNRGENSCKATGQVCHALCSPEGCWGPEPRDCVSCRNVSRGRECVDKCNLLEGEPREFVENSECIQCHPECLPQAMNITCTGRGPDNCIQCAHYIDGPHCVKTCPAGVMGENNTLVWKYADAGHVCHLCHPNCTYGCTGPGLEGCPTNGPKIPSIATGMVGALLLLLVVALGIGLFM

SEQ ID NO: 41 - DNA, 9400 bp, synthetic construct
  misc_feature 1..9400: note = Synthetic
  source 1..9400: mol_type = other DNA
gttagaccagatctgagcctgggagctctctggctaactagggaacccactgcttaagcctcaataaagcttgccttgagtgcttcaagtagtgtgtgcccgtctgttgtgtgactctggtaactagagatccctcagacccttttagtcagtgtggaaaatctctagcagtggcgcccgaacagggacttgaaagcgaaagggaaaccagaggagctctctcgacgcaggactcggcttgctgaagcgcgcacggcaagaggcgaggggcggcgactggtgagtacgccaaaaattttgactagcggaggctagaaggagagagatgggtgcgagagcgtcagtattaagcgggggagaattagatcgatgggaaaaaattcggttaaggccagggggaaagaaaaaatataaattaaaacatatagtatgggcaagcagggagctagaacgattcgcagttaatcctggcctgttagaaacatcagaaggctgtagacaaatactgggacagctacaaccatcccttcagacaggatcagaagaacttagatcattatataatacagtagcaaccctctattgtgtgcatcaaaggatagagataaaagacaccaaggaagctttagacaagatagaggaagagcaaaacaaaagtaagaaaaaagcacagcaagcagcagctgacacaggacacagcaatcaggtcagccaaaattaccctatagtgcagaacatccaggggcaaatggtacatcaggccatatcacctagaactttaaatgcatgggtaaaagtagtagaagagaaggctttcagcccagaagtgatacccatgttttcagcattatcagaaggagccaccccacaagatttaaacaccatgctaaacacagtggggggacatcaagcagccatgcaaatgttaaaagagaccatcaatgaggaagctgcaggcaaagagaagagtggtgcagagagaaaaaagagcagtgggaataggagctttgttccttgggttcttgggagcagcaggaagcactatgggcgcagcgtcaatgacgctgacggtacaggccagacaattattgtctggtatagtgcagcagcagaacaatttgctgagggctattgaggcgcaacagcatctgttgcaactcacagtctggggcatcaagcagctccaggcaagaatcctggctgtggaaagatacctaaaggatcaacagctcctggggatttggggttgctctggaaaactcatttgcaccactgctgtgccttggatctacaaatggcagtattcatccacaattttaaaagaaaaggggggattggggggtacagtgcaggggaaagaatagtagacataatagcaacagacatacaaactaaagaattacaaaaacaaattacaaaaattcaaaattttcgggtttattacagggacagcagagatccagtttggggatcaattgcatgaagaatctgcttagggttaggcgttttgcgctgcttcgcgaggatctgcgatcgctccggtgcccgtcagtgggcagagcgcacatcgcccacagtccccgagaagttggggggaggggtcggcaattgaaccggtgcctagagaaggtggcgcggggtaaactgggaaagtgatgtcgtgtactggctccgcctttttcccgagggtgggggagaaccgtatataagtgcagtagtcgccgtgaacgttctttttcgcaacgggtttgccgccagaacacagctgaagcttcgaggggctcgcatctctccttcacgcgcccgccgccctacctgaggccgccatccacgccggttgagtcgcgttctgccgcctcccgcctgtggtgcctcctgaactgcgtccgccgtctaggtaagtttaaagctcaggtcgagaccgggcctttgtccggcgctcccttggagcctacctagactcagccggctctccacgctttgcctgaccctgcttgctcaactctacgtctttgtttcgttttctgttctgcgccgttacagatccaagctgtgaccggcgcctacggctagcgaattcctcgaggccaccatgctgctgctggtgacaagcctgctgctgtgcgagctgccccaccccgcctttctgctgatcccccaggaacagctcgtcgaaagcggcggcagactggtgacacctggcggcagcctgaccctgagctgcaaggccagcggcttcgacttcagcgcctactacatgagctgggtccgccaggcccctggcaagggactggaatggatcgccaccatctaccccagcagcggcaagacctactacgccacctgggtgaacggacggttcaccatctccagcgacaacgcccagaacaccgtggacctgcagatgaacagcctgacagccgccgaccgggccacctacttttgcgccagagacagctacgccgacgacggcgccctgttcaacatctggggccctggcaccctggtgacaatctctagcggcggaggcggatctggtggcggaggaagtggcggcggaggatctgagctggtgctgacccagagcccctctgtgtctgctgccctgggaagccctgccaagatcacctgtaccctgagcagcgcccacaagaccgacaccatcgactggtatcagcagctgcagggcgaggcccccagatacctgatgcaggtgcagagcgacggcagctacaccaagaggccaggcgtgcccgaccggttcagcggatctagctctggcgccgaccgctacctgatcatccccagcgtgcaggccgatgacgaggccgattactactgtggcgccgactacatcggcggctacgtgttcggcggaggcacccagctgaccgtgaccggcgagtctaagtacggaccgccctgccccccttgccctatgttctgggtgctggtggtggtgggcggggtgctggcctgctacagcctgctggtgacagtggccttcatcatcttttgggtgaaacggggcagaaagaaactcctgtatatattcaaacaaccatttatgagaccagtacaaactactcaagaggaagatggctgtagctgccgatttccagaagaagaagaaggaggatgtgaactgcgggtgaagttcagcagaagcgccgacgcccctgcctaccagcagggccagaatcagctgtacaacgagctgaacctgggcagaagggaagagtacgacgtcctggataagcggagaggccgggaccctgagatgggcggcaagcctcggcggaagaacccccaggaaggcctgtataacgaactgcagaaagacaagatggccgaggcctacagcgagatcggcatgaagggcgagcggaggcggggcaagggccacgacggcctgtatcagggcctgtccaccgccaccaaggatacctacgacgccctgcacatgcaggccctgcccccaaggctcgagggcggcggagagggcagaggaagtcttctaacatgcggtgacgtggaggagaatcccggccctaggatgcttctcctggtgacaagccttctgctctgtgagttaccacacccagcattcctcctgatcccacgcaaagtgtgtaacggaataggtattggtgaatttaaagactcactctccataaatgctacgaatattaaacacttcaaaaactgcacctccatcagtggcgatctccacatcctgccggtggcatttaggggtgactccttcacacatactcctcctctggatccacaggaactggatattctgaaaaccgtaaaggaaatcacagggtttttgctgattcaggcttggcctgaaaacaggacggacctccatgcctttgagaacctagaaatcatacgcggcaggaccaagcaacatggtcagttttctcttgcagtcgtcagcctgaacataacatccttgggattacgctccctcaaggagataagtgatggagatgtgataatttcaggaaacaaaaatttgtgctatgcaaatacaataaactggaaaaaactgtttgggacctccggtcagaaaaccaaaattataagcaacagaggtgaaaacagctgcaaggccacaggccaggtctgccatgccttgtgctcccccgagggctgctggggcccggagcccagggactgcgtctcttgccggaatgtcagccgaggcagggaatgcgtggacaagtgcaaccttctggagggtgagccaagggagtttgtggagaactctgagtgcatacagtgccacccagagtgcctgcctcaggccatgaacatcacctgcacaggacggggaccagacaactgtatccagtgtgcccactacattgacggcccccactgcgtcaagacctgcccggcaggagtcatgggagaaaacaacaccctggtctggaagtacgcagacgccggccatgtgtgccacctgtgccatccaaactgcacctacggatgcactgggccaggtcttgaaggctgtccaacgaatgggcctaagatcccgtccatcgccactgggatggtgggggccctcctcttgctgctggtggtggccctggggatcggcctcttcatgtgagcggccgctctagacccgggctgcaggaattcgatatcaagcttatcgataatcaacctctggattacaaaatttgtgaaagattgactggtattcttaactatgttgctccttttacgctatgtggatacgctgctttaatgcctttgtatcatgctattgcttcccgtatggctttcattttctcctccttgtataaatcctggttgctgtctctttatgaggagttgtggcccgttgtcaggcaacgtggcgtggtgtgcactgtgtttgctgacgcaacccccactggttggggcattgccaccacctgtcagctcctttccgggactttcgctttccccctccctattgccacggcggaactcatcgccgcctgccttgcccgctgctggacaggggctcggctgttgggcactgacaattccgtggtgttgtcggggaaatcatcgtcctttccttggctgctcgcctgtgttgccacctggattctgcgcgggacgtccttctgctacgtcccttcggccctcaatccagcggaccttccttcccgcggcctgctgccggctctgcggcctcttccgcgtcttcgccttcgccctcagacgagtcggatctccctttgggccgcctccccgcatcgataccgtcgactagccgtacctttaagaccaatgacttacaaggcagctgtagatcttagccactttttaaaagaaaaggggggactggaagggctaattcactcccaaagaagacaagatctgctttttgcctgtactgggtctctctggttagaccagatctgagcctgggagctctctggctaactagggaacccactgcttaagcctcaataaagcttgccttgagtgcttcaagtagtgtgtgcccgtctgttgtgtgactctggtaactagagatccctcagacccttttagtcagtgtggaaaatctctagcagaattcgatatcaagcttatcgataccgtcgacctcgagggggggcccggtacccaattcgccctatagtgagtcgtattacaattcactggccgtcgttttacaacgtcgtgactgggaaaaccctggcgttacccaacttaatcgccttgcagcacatccccctttcgccagctggcgtaatagcgaagaggcccgcaccgatcgcccttcccaacagttgcgcagcctgaatggcgaatggaaattgtaagcgttaatattttgttaaaattcgcgttaaatttttgttaaatcagctcattttttaaccaataggccgaaatcggcaaaatcccttataaatcaaaagaatagaccgagatagggttgagtgttgttccagtttggaacaagagtccactattaaagaacgtggactccaacgtcaaagggcgaaaaaccgtctatcagggcgatggcccactacgtgaaccatcaccctaatcaagttttttggggtcgaggtgccgtaaagcactaaatcggaaccctaaagggagcccccgatttagagcttgacggggaaagccggcgaacgtggcgagaaaggaagggaagaaagcgaaaggagcgggcgctagggcgctggcaagtgtagcggtcacgctgcgcgtaaccaccacacccgccgcgcttaatgcgccgctacagggcgcgtcaggtggcacttttcggggaaatgtgcgcggaacccctatttgtttatttttctaaatacattcaaatatgtatccgctcatgagacaataaccctgataaatgcttcaataatattgaaaaaggaagagtatgagtattcaacatttccgtgtcgcccttattcccttttttgcggcattttgccttcctgtttttgctcacccagaaacgctggtgaaagtaaaagatgctgaagatcagttgggtgcacgagtgggttacatcgaactggatctcaacagcggtaagatccttgagagttttcgccccgaagaacgttttccaatgatgagcacttttaaagttctgctatgtggcgcggtattatcccgtattgacgccgggcaagagcaactcggtcgccgcatacactattctcagaatgacttggttgagtactcaccagtcacagaaaagcatcttacggatggcatgacagtaagagaattatgcagtgctgccataaccatgagtgataacactgcggccaacttacttctgacaacgatcggaggaccgaaggagctaaccgcttttttgcacaacatgggggatcatgtaactcgccttgatcgttgggaaccggagctgaatgaagccataccaaacgacgagcgtgacaccacgatgcctgtagcaatggcaacaacgttgcgcaaactattaactggcgaactacttactctagcttcccggcaacaattaatagactggatggaggcggataaagttgcaggaccacttctgcgctcggcccttccggctggctggtttattgctgataaatctggagccggtgagcgtgggtctcgcggtatcattgcagcactggggccagatggtaagccctcccgtatcgtagttatctacacgacggggagtcaggcaactatggatgaacgaaatagacagatcgctgagataggtgcctcactgattaagcattggtaactgtcagaccaagtttactcatatatactttagattgatttaaaacttcatttttaatttaaaaggatctaggtgaagatcctttttgataatctcatgaccaaaatcccttaacgtgagttttcgttccactgagcgtcagaccccgtagaaaagatcaaaggatcttcttgagatcctttttttctgcgcgtaatctgctgcttgcaaacaaaaaaaccaccgctaccagcggtggtttgtttgccggatcaagagctaccaactctttttccgaaggtaactggcttcagcagagcgcagataccaaatactgttcttctagtgtagccgtagttaggccaccacttcaagaactctgtagcaccgcctacatacctcgctctgctaatcctgttaccagtggctgctgccagtggcgataagtcgtgtcttaccgggttggactcaagacgatagttaccggataaggcgcagcggtcgggctgaacggggggttcgtgcacacagcccagcttggagcgaacgacctacaccgaactgagatacctacagcgtgagctatgagaaagcgccacgcttcccgaagggagaaaggcggacaggtatccggtaagcggcagggtcggaacaggagagcgcacgagggagcttccagggggaaacgcctggtatctttatagtcctgtcgggtttcgccacctctgacttgagcgtcgatttttgtgatgctcgtcaggggggcggagcctatggaaaaacgccagcaacgcggcctttttacggttcctggccttttgctggccttttgctcacatgttctttcctgcgttatcccctgattctgtggataaccgtattaccgcctttgagtgagctgataccgctcgccgcagccgaacgaccgagcgcagcgagtcagtgagcgaggaagcggaagagcgcccaatacgcaaaccgcctctccccgcgcgttggccgattcattaatgcagctggcacgacaggtttcccgactggaaagcgggcagtgagcgcaacgcaattaatgtgagttagctcactcattaggcaccccaggctttacactttatgcttccggctcgtatgttgtgtggaattgtgagcggataacaatttcacacaggaaacagctatgaccatgattacgccaagctcgaaattaaccctcactaaagggaacaaaagctggagctccaccgcggtggcggcctcgaggtcgagatccggtcgaccagcaaccatagtcccgcccctaactccgcccatcccgcccctaactccgcccagttccgcccattctccgccccatggctgactaattttttttatttatgcagaggccgaggccgcctcggcctctgagctattccagaagtagtgaggaggcttttttggaggcctaggcttttgcaaaaagcttcgacggtatcgattggctcatgtccaacattaccgccatgttgacattgattattgactagttattaatagtaatcaattacggggtcattagttcatagcccatatatggagttccgcgttacataacttacggtaaatggcccgcctggctgaccgcccaacgacccccgcccattgacgtcaataatgacgtatgttcccatagtaacgccaatagggactttccattgacgtcaatgggtggagtatttacggtaaactgcccacttggcagtacatcaagtgtatcatatgccaagtacgccccctattgacgtcaatgacggtaaatggcccgcctggcattatgcccagtacatgaccttatgggactttcctacttggcagtacatctacgtattagtcatcgctattaccatggtgatgcggttttggcagtacatcaatgggcgtggatagcggtttgactcacggggatttccaagtctccaccccattgacgtcaatgggagtttgttttggcaccaaaatcaacgggactttccaaaatgtcgtaacaactccgccccattgacgcaaatgggcggtaggcgtgtacggaattcggagtggcgagccctcagatcctgcatataagcagctgctttttgcctgtactgggtctctctg

SEQ ID NO: 42 - protein, 845 aa, synthetic construct
  REGION 1..845: note = Synthetic
MLLLVTSLLLCELPHPAFLLIPQEQLVESGGRLVTPGGSLTLSCKASGFDFSAYYMSWVRQAPGKGLEWIATIYPSSGKTYYATWVNGRFTISSDNAQNTVDLQMNSLTAADRATYFCARDSYADDGALFNIWGPGTLVTISSGGGGSGGGGSGGGGSELVLTQSPSVSAALGSPAKITCTLSSAHKTDTIDWYQQLQGEAPRYLMQVQSDGSYTKRPGVPDRFSGSSSGADRYLIIPSVQADDEADYYCGADYIGGYVFGGGTQLTVTGESKYGPPCPPCPMFWVLVVVGGVLACYSLLVTVAFIIFWVKRGRKKLLYIFKQPFMRPVQTTQEEDGCSCRFPEEEEGGCELRVKFSRSADAPAYQQGQNQLYNELNLGRREEYDVLDKRRGRDPEMGGKPRRKNPQEGLYNELQKDKMAEAYSEIGMKGERRRGKGHDGLYQGLSTATKDTYDALHMQALPPRLEGGGEGRGSLLTCGDVEENPGPRMLLLVTSLLLCELPHPAFLLIPRKVCNGIGIGEFKDSLSINATNIKHFKNCTSISGDLHILPVAFRGDSFTHTPPLDPQELDILKTVKEITGFLLIQAWPENRTDLHAFENLEIIRGRTKQHGQFSLAVVSLNITSLGLRSLKEISDGDVIISGNKNLCYANTINWKKLFGTSGQKTKIISNRGENSCKATGQVCHALCSPEGCWGPEPRDCVSCRNVSRGRECVDKCNLLEGEPREFVENSECIQCHPECLPQAMNITCTGRGPDNCIQCAHYIDGPHCVKTCPAGVMGENNTLVWKYADAGHVCHLCHPNCTYGCTGPGLEGCPTNGPKIPSIATGMVGALLLLLVVALGIGLFM

SEQ ID NO: 43 - DNA, 10015 bp, synthetic construct
  misc_feature 1..10015: note = Synthetic
  source 1..10015: mol_type = other DNA
gttagaccagatctgagcctgggagctctctggctaactagggaacccactgcttaagcctcaataaagcttgccttgagtgcttcaagtagtgtgtgcccgtctgttgtgtgactctggtaactagagatccctcagacccttttagtcagtgtggaaaatctctagcagtggcgcccgaacagggacttgaaagcgaaagggaaaccagaggagctctctcgacgcaggactcggcttgctgaagcgcgcacggcaagaggcgaggggcggcgactggtgagtacgccaaaaattttgactagcggaggctagaaggagagagatgggtgcgagagcgtcagtattaagcgggggagaattagatcgatgggaaaaaattcggttaaggccagggggaaagaaaaaatataaattaaaacatatagtatgggcaagcagggagctagaacgattcgcagttaatcctggcctgttagaaacatcagaaggctgtagacaaatactgggacagctacaaccatcccttcagacaggatcagaagaacttagatcattatataatacagtagcaaccctctattgtgtgcatcaaaggatagagataaaagacaccaaggaagctttagacaagatagaggaagagcaaaacaaaagtaagaaaaaagcacagcaagcagcagctgacacaggacacagcaatcaggtcagccaaaattaccctatagtgcagaacatccaggggcaaatggtacatcaggccatatcacctagaactttaaatgcatgggtaaaagtagtagaagagaaggctttcagcccagaagtgatacccatgttttcagcattatcagaaggagccaccccacaagatttaaacaccatgctaaacacagtggggggacatcaagcagccatgcaaatgttaaaagagaccatcaatgaggaagctgcaggcaaagagaagagtggtgcagagagaaaaaagagcagtgggaataggagctttgttccttgggttcttgggagcagcaggaagcactatgggcgcagcgtcaatgacgctgacggtacaggccagacaattattgtctggtatagtgcagcagcagaacaatttgctgagggctattgaggcgcaacagcatctgttgcaactcacagtctggggcatcaagcagctccaggcaagaatcctggctgtggaaagatacctaaaggatcaacagctcctggggatttggggttgctctggaaaactcatttgcaccactgctgtgccttggatctacaaatggcagtattcatccacaattttaaaagaaaaggggggattggggggtacagtgcaggggaaagaatagtagacataatagcaacagacatacaaactaaagaattacaaaaacaaattacaaaaattcaaaattttcgggtttattacagggacagcagagatccagtttggggatcaattgcatgaagaatctgcttagggttaggcgttttgcgctgcttcgcgaggatctgcgatcgctccggtgcccgtcagtgggcagagcgcacatcgcccacagtccccgagaagttggggggaggggtcggcaattgaaccggtgcctagagaaggtggcgcggggtaaactgggaaagtgatgtcgtgtactggctccgcctttttcccgagggtgggggagaaccgtatataagtgcagtagtcgccgtgaacgttctttttcgcaacgggtttgccgccagaacacagctgaagcttcgaggggctcgcatctctccttcacgcgcccgccgccctacctgaggccgccatccacgccggttgagtcgcgttctgccgcctcccgcctgtggtgcctcctgaactgcgtccgccgtctaggtaagtttaaagctcaggtcgagaccgggcctttgtccggcgctcccttggagcctacctagactcagccggctctccacgctttgcctgaccctgcttgctcaactctacgtctttgtttcgttttctgttctgcgccgttacagatccaagctgtgaccggcgcctacggctagcgaattcgccaccatgctgctgctggtgacaagcctgctgctgtgcgagctgccccaccccgcctttctgctgatcccccagagcgtgaaagagtccgagggcgacctggtcacaccagccggcaacctgaccctgacctgtaccgccagcggcagcgacatcaacgactaccccatctcttgggtccgccaggctcctggcaagggactggaatggatcggcttcatcaacagcggcggcagcacttggtacgccagctgggtcaaaggccggttcaccatcagccggaccagcaccaccgtggacctgaagatgacaagcctgaccaccgacgacaccgccacctacttttgcgccagaggctacagcacctactacggcgacttcaacatctggggccctggcaccctggtcacaatctctagcggcggaggcggcagcggaggtggaggaagtggcggcggaggatccgagctggtcatgacccagacccccagcagcacatctggcgccgtgggcggcaccgtgaccatcaattgccaggccagccagagcatcgacagcaacctggcctggttccagcagaagcccggccagccccccaccctgctgatctacagagcctccaacctggccagcggcgtgccaagcagattcagcggcagcagatctggcaccgagtacaccctgaccatctccggcgtgcagagagaggacgccgctacctattactgcctgggcggcgtgggcaacgtgtcctacagaaccagcttcggcggaggtactgaggtggtcgtcaaatacggaccgccctgccccccttgccctgcccccgagttcctgggcggacccagcgtgttcctgttcccccccaagcccaaggacaccctgatgatcagccggacccccgaggtgacctgcgtggtggtggacgtgagccaggaagatcccgaggtccagttcaattggtacgtggacggcgtggaagtgcacaacgccaagaccaagcccagagaggaacagttcaacagcacctaccgggtggtgtctgtgctgaccgtgctgcaccaggactggctgaacggcaaagaatacaagtgcaaggtgtccaacaagggcctgcccagcagcatcgaaaagaccatcagcaaggccaagggccagcctcgcgagccccaggtgtacaccctgcctccctcccaggaagagatgaccaagaaccaggtgtccctgacctgcctggtgaagggcttctaccccagcgacatcgccgtggagtgggagagcaacggccagcctgagaacaactacaagaccacccctcccgtgctggacagcgacggcagcttcttcctgtacagccggctgaccgtggacaagagccggtggcaggaaggcaacgtctttagctgcagcgtgatgcacgaggccctgcacaaccactacacccagaagagcctgagcctgtccctgggcaagatgttctgggtgctggtggtggtgggcggggtgctggcctgctacagcctgctggtgacagtggccttcatcatcttttgggtgaaacggggcagaaagaaactcctgtatatattcaaacaaccatttatgagaccagtacaaactactcaagaggaagatggctgtagctgccgatttccagaagaagaagaaggaggatgtgaactgcgggtgaagttcagcagaagcgccgacgcccctgcctaccagcagggccagaatcagctgtacaacgagctgaacctgggcagaagggaagagtacgacgtcctggataagcggagaggccgggaccctgagatgggcggcaagcctcggcggaagaacccccaggaaggcctgtataacgaactgcagaaagacaagatggccgaggcctacagcgagatcggcatgaagggcgagcggaggcggggcaagggccacgacggcctgtatcagggcctgtccaccgccaccaaggatacctacgacgccctgcacatgcaggccctgcccccaaggctcgagggcggcggagagggcagaggaagtcttctaacatgcggtgacgtggaggagaatcccggccctaggatgcttctcctggtgacaagccttctgctctgtgagttaccacacccagcattcctcctgatcccacgcaaagtgtgtaacggaataggtattggtgaatttaaagactcactctccataaatgctacgaatattaaacacttcaaaaactgcacctccatcagtggcgatctccacatcctgccggtggcatttaggggtgactccttcacacatactcctcctctggatccacaggaactggatattctgaaaaccgtaaaggaaatcacagggtttttgctgattcaggcttggcctgaaaacaggacggacctccatgcctttgagaacctagaaatcatacgcggcaggaccaagcaacatggtcagttttctcttgcagtcgtcagcctgaacataacatccttgggattacgctccctcaaggagataagtgatggagatgtgataatttcaggaaacaaaaatttgtgctatgcaaatacaataaactggaaaaaactgtttgggacctccggtcagaaaaccaaaattataagcaacagaggtgaaaacagctgcaaggccacaggccaggtctgccatgccttgtgctcccccgagggctgctggggcccggagcccagggactgcgtctcttgccggaatgtcagccgaggcagggaatgcgtggacaagtgcaaccttctggagggtgagccaagggagtttgtggagaactctgagtgcatacagtgccacccagagtgcctgcctcaggccatgaacatcacctgcacaggacggggaccagacaactgtatccagtgtgcccactacattgacggcccccactgcgtcaagacctgcccggcaggagtcatgggagaaaacaacaccctggtctggaagtacgcagacgccggccatgtgtgccacctgtgccatccaaactgcacctacggatgcactgggccaggtcttgaaggctgtccaacgaatgggcctaagatcccgtccatcgccactgggatggtgggggccctcctcttgctgctggtggtggccctggggatcggcctcttcatgtgagcggccgctctagacccgggctgcaggaattcgatatcaagcttatcgataatcaacctctggattacaaaatttgtgaaagattgactggtattcttaactatgttgctccttttacgctatgtggatacgctgctttaatgcctttgtatcatgctattgcttcccgtatggctttcattttctcctccttgtataaatcctggttgctgtctctttatgaggagttgtggcccgttgtcaggcaacgtggcgtggtgtgcactgtgtttgctgacgcaacccccactggttggggcattgccaccacctgtcagctcctttccgggactttcgctttccccctccctattgccacggcggaactcatcgccgcctgccttgcccgctgctggacaggggctcggctgttgggcactgacaattccgtggtgttgtcggggaaatcatcgtcctttccttggctgctcgcctgtgttgccacctggattctgcgcgggacgtccttctgctacgtcccttcggccctcaatccagcggaccttccttcccgcggcctgctgccggctctgcggcctcttccgcgtcttcgccttcgccctcagacgagtcggatctccctttgggccgcctccccgcatcgataccgtcgactagccgtacctttaagaccaatgacttacaaggcagctgtagatcttagccactttttaaaagaaaaggggggactggaagggctaattcactcccaaagaagacaagatctgctttttgcctgtactgggtctctctggttagaccagatctgagcctgggagctctctggctaactagggaacccactgcttaagcctcaataaagcttgccttgagtgcttcaagtagtgtgtgcccgtctgttgtgtgactctggtaactagagatccctcagacccttttagtcagtgtggaaaatctctagcagaattcgatatcaagcttatcgataccgtcgacctcgagggggggcccggtacccaattcgccctatagtgagtcgtattacaattcactggccgtcgttttacaacgtcgtgactgggaaaaccctggcgttacccaacttaatcgccttgcagcacatccccctttcgccagctggcgtaatagcgaagaggcccgcaccgatcgcccttcccaacagttgcgcagcctgaatggcgaatggaaattgtaagcgttaatattttgttaaaattcgcgttaaatttttgttaaatcagctcattttttaaccaataggccgaaatcggcaaaatcccttataaatcaaaagaatagaccgagatagggttgagtgttgttccagtttggaacaagagtccactattaaagaacgtggactccaacgtcaaagggcgaaaaaccgtctatcagggcgatggcccactacgtgaaccatcaccctaatcaagttttttggggtcgaggtgccgtaaagcactaaatcggaaccctaaagggagcccccgatttagagcttgacggggaaagccggcgaacgtggcgagaaaggaagggaagaaagcgaaaggagcgggcgctagggcgctggcaagtgtagcggtcacgctgcgcgtaaccaccacacccgccgcgcttaatgcgccgctacagggcgcgtcaggtggcacttttcggggaaatgtgcgcggaacccctatttgtttatttttctaaatacattcaaatatgtatccgctcatgagacaataaccctgataaatgcttcaataatattgaaaaaggaagagtatgagtattcaacatttccgtgtcgcccttattcccttttttgcggcattttgccttcctgtttttgctcacccagaaacgctggtgaaagtaaaagatgctgaagatcagttgggtgcacgagtgggttacatcgaactggatctcaacagcggtaagatccttgagagttttcgccccgaagaacgttttccaatgatgagcacttttaaagttctgctatgtggcgcggtattatcccgtattgacgccgggcaagagcaactcggtcgccgcatacactattctcagaatgacttggttgagtactcaccagtcacagaaaagcatcttacggatggcatgacagtaagagaattatgcagtgctgccataaccatgagtgataacactgcggccaacttacttctgacaacgatcggaggaccgaaggagctaaccgcttttttgcacaacatgggggatcatgtaactcgccttgatcgttgggaaccggagctgaatgaagccataccaaacgacgagcgtgacaccacgatgcctgtagcaatggcaacaacgttgcgcaaactattaactggcgaactacttactctagcttcccggcaacaattaatagactggatggaggcggataaagttgcaggaccacttctgcgctcggcccttccggctggctggtttattgctgataaatctggagccggtgagcgtgggtctcgcggtatcattgcagcactggggccagatggtaagccctcccgtatcgtagttatctacacgacggggagtcaggcaactatggatgaacgaaatagacagatcgctgagataggtgcctcactgattaagcattggtaactgtcagaccaagtttactcatatatactttagattgatttaaaacttcatttttaatttaaaaggatctaggtgaagatcctttttgataatctcatgaccaaaatcccttaacgtgagttttcgttccactgagcgtcagaccccgtagaaaagatcaaaggatcttcttgagatcctttttttctgcgcgtaatctgctgcttgcaaacaaaaaaaccaccgctaccagcggtggtttgtttgccggatcaagagctaccaactctttttccgaaggtaactggcttcagcagagcgcagataccaaatactgttcttctagtgtagccgtagttaggccaccacttcaagaactctgtagcaccgcctacatacctcgctctgctaatcctgttaccagtggctgctgccagtggcgataagtcgtgtcttaccgggttggactcaagacgatagttaccggataaggcgcagcggtcgggctgaacggggggttcgtgcacacagcccagcttggagcgaacgacctacaccgaactgagatacctacagcgtgagctatgagaaagcgccacgcttcccgaagggagaaaggcggacaggtatccggtaagcggcagggtcggaacaggagagcgcacgagggagcttccagggggaaacgcctggtatctttatagtcctgtcgggtttcgccacctctgacttgagcgtcgatttttgtgatgctcgtcaggggggcggagcctatggaaaaacgccagcaacgcggcctttttacggttcctggccttttgctggccttttgctcacatgttctttcctgcgttatcccctgattctgtggataaccgtattaccgcctttgagtgagctgataccgctcgccgcagccgaacgaccgagcgcagcgagtcagtgagcgaggaagcggaagagcgcccaatacgcaaaccgcctctccccgcgcgttggccgattcattaatgcagctggcacgacaggtttcccgactggaaagcgggcagtgagcgcaacgcaattaatgtgagttagctcactcattaggcaccccaggctttacactttatgcttccggctcgtatgttgtgtggaattgtgagcggataacaatttcacacaggaaacagctatgaccatgattacgccaagctcgaaattaaccctcactaaagggaacaaaagctggagctccaccgcggtggcggcctcgaggtcgagatccggtcgaccagcaaccatagtcccgcccctaactccgcccatcccgcccctaactccgcccagttccgcccattctccgccccatggctgactaattttttttatttatgcagaggccgaggccgcctcggcctctgagctattccagaagtagtgaggaggcttttttggaggcctaggcttttgcaaaaagcttcgacggtatcgattggctcatgtccaacattaccgccatgttgacattgattattgactagttattaatagtaatcaattacggggtcattagttcatagcccatatatggagttccgcgttacataacttacggtaaatggcccgcctggctgaccgcccaacgacccccgcccattgacgtcaataatgacgtatgttcccatagtaacgccaatagggactttccattgacgtcaatgggtggagtatttacggtaaactgcccacttggcagtacatcaagtgtatcatatgccaagtacgccccctattgacgtcaatgacggtaaatggcccgcctggcattatgcccagtacatgaccttatgggactttcctacttggcagtacatctacgtattagtcatcgctattaccatggtgatgcggttttggcagtacatcaatgggcgtggatagcggtttgactcacggggatttccaagtctccaccccattgacgtcaatgggagtttgttttggcaccaaaatcaacgggactttccaaaatgtcgtaacaactccgccccattgacgcaaatgggcggtaggcgtgtacggaattcggagtggcgagccctcagatcctgcatataagcagctgctttttgcctgtactgggtctctctg

SEQ ID NO: 44 - protein, 1055 aa, synthetic construct [sequence omitted]

SEQ ID NO: 45 - DNA, 10015 bp, synthetic construct; identical to SEQ ID NO: 43
  misc_feature 1..10015: note = Synthetic
  source 1..10015: mol_type = other DNA

SEQ ID NO: 46 - protein, 945 aa, synthetic construct
  REGION 1..945: note = Synthetic
MLLLVTSLLLCELPHPAFLLIPQSVKESEGDLVTPAGNLTLTCTASGSDINDYPISWVRQAPGKGLEWIGFINSGGSTWYASWVKGRFTISRTSTTVDLKMTSLTTDDTATYFCARGYSTYYGDFNIWGPGTLVTISSGGGGSGGGGSGGGGSELVMTQTPSSTSGAVGGTVTINCQASQSIDSNLAWFQQKPGQPPTLLIYRASNLASGVPSRFSGSRSGTEYTLTISGVQREDAATYYCLGGVGNVSYRTSFGGGTEVVVKESKYGPPCPPCPGQPREPQVYTLPPSQEEMTKNQVSLTCLVKGFYPSDIAVEWESNGQPENNYKTTPPVLDSDGSFFLYSRLTVDKSRWQEGNVFSCSVMHEALHNHYTQKSLSLSLGKMFWVLVVVGGVLACYSLLVTVAFIIFWVKRGRKKLLYIFKQPFMRPVQTTQEEDGCSCRFPEEEEGGCELRVKFSRSADAPAYQQGQNQLYNELNLGRREEYDVLDKRRGRDPEMGGKPRRKNPQEGLYNELQKDKMAEAYSEIGMKGERRRGKGHDGLYQGLSTATKDTYDALHMQALPPRLEGGGEGRGSLLTCGDVEENPGPRMLLLVTSLLLCELPHPAFLLIPRKVCNGIGIGEFKDSLSINATNIKHFKNCTSISGDLHILPVAFRGDSFTHTPPLDPQELDILKTVKEITGFLLIQAWPENRTDLHAFENLEIIRGRTKQHGQFSLAVVSLNITSLGLRSLKEISDGDVIISGNKNLCYANTINWKKLFGTSGQKTKIISNRGENSCKATGQVCHALCSPEGCWGPEPRDCVSCRNVSRGRECVDKCNLLEGEPREFVENSECIQCHPECLPQAMNITCTGRGPDNCIQCAHYIDGPHCVKTCPAGVMGENNTLVWKYADAGHVCHLCHPNCTYGCTGPGLEGCPTNGPKIPSIATGMVGALLLLLVVALGIGLFM

SEQ ID NO: 47 - DNA, 9685 bp, synthetic construct
  misc_feature 1..9685: note = Synthetic
  source 1..9685: mol_type = other DNA
gttagaccagatctgagcctgggagctctctggctaactagggaacccactgcttaagcctcaataaagcttgccttgagtgcttcaagtagtgtgtgcccgtctgttgtgtgactctggtaactagagatccctcagacccttttagtcagtgtggaaaatctctagcagtggcgcccgaacagggacttgaaagcgaaagggaaaccagaggagctctctcgacgcaggactcggcttgctgaagcgcgcacggcaagaggcgaggggcggcgactggtgagtacgccaaaaattttgactagcggaggctagaaggagagagatgggtgcgagagcgtcagtattaagcgggggagaattagatcgatgggaaaaaattcggttaaggccagggggaaagaaaaaatataaattaaaacatatagtatgggcaagcagggagctagaacgattcgcagttaatcctggcctgttagaaacatcagaaggctgtagacaaatactgggacagctacaaccatcccttcagacaggatcagaagaacttagatcattatataatacagtagcaaccctctattgtgtgcatcaaaggatagagataaaagacaccaaggaagctttagacaagatagaggaagagcaaaacaaaagtaagaaaaaagcacagcaagcagcagctgacacaggacacagcaatcaggtcagccaaaattaccctatagtgcagaacatccaggggcaaatggtacatcaggccatatcacctagaactttaaatgcatgggtaaaagtagtagaagagaaggctttcagcccagaagtgatacccatgttttcagcattatcagaaggagccaccccacaagatttaaacaccatgctaaacacagtggggggacatcaagcagccatgcaaatgttaaaagagaccatcaatgaggaagctgcaggcaaagagaagagtggtgcagagagaaaaaagagcagtgggaataggagctttgttccttgggttcttgggagcagcaggaagcactatgggcgcagcgtcaatgacgctgacggtacaggccagacaattattgtctggtatagtgcagcagcagaacaatttgctgagggctattgaggcgcaacagcatctgttgcaactcacagtctggggcatcaagcagctccaggcaagaatcctggctgtggaaagatacctaaaggatcaacagctcctggggatttggggttgctctggaaaactcatttgcaccactgctgtgccttggatctacaaatggcagtattcatccacaattttaaaagaaaaggggggattggggggtacagtgcaggggaaagaatagtagacataatagcaacagacatacaaactaaagaattacaaaaacaaattacaaaaattcaaaattttcgggtttattacagggacagcagagatccagtttggggatcaattgcatgaagaatctgcttagggttaggcgttttgcgctgcttcgcgaggatctgcgatcgctccggtgcccgtcagtgggcagagcgcacatcgcccacagtccccgagaagttggggggaggggtcggcaattgaaccggtgcctagagaaggtggcgcggggtaaactgggaaagtgatgtcgtgtactggctccgcctttttcccgagggtgggggagaaccgtatataagtgcagtagtcgccgtgaacgttctttttcgcaacgggtttgccgccagaacacagctgaagcttcgaggggctcgcatctctccttcacgcgcccgccgccctacctgaggccgccatccacgccggttgagtcgcgttctgccgcctcccgcctgtggtgcctcctgaactgcgtccgccgtctaggtaagtttaaagctcaggtcgagaccgggcctttgtccggcgctcccttggagcctacctagactcagccggctctccacgctttgcctgaccctgcttgctcaactctacgtctttgtttcgttttctgttctgcgccgttacagatccaagctgtgaccggcgcctacggctagcgaattcgccaccatgctgctgctggtgacaagcctgctgctgtgcgagctgccccaccccgcctttctgctgatcccccagagcgtgaaagagtccgagggcgacctggtcacaccagccggcaacctgaccctgacctgtaccgccagcggcagcgacatcaacgactaccccatctcttgggtccgccaggctcctggcaagggactggaatggatcggcttcatcaacagcggcggcagcacttggtacgccagctgggtcaaaggccggttcaccatcagccggaccagcaccaccgtggacctgaagatgacaagcctgaccaccgacgacaccgccacctacttttgcgccagaggctacagcacctactacggcgacttcaacatctggggccctggcaccctggtcacaatctctagcggcggaggcggcagcggaggtggaggaagtggcggcggaggatccgagctggtcatgacccagacccccagcagcacatctggcgccgtgggcggcaccgtgaccatcaattgccaggccagccagagcatcgacagcaacctggcctggttccagcagaagcccggccagccccccaccctgctgatctacagagcctccaacctggccagcggcgtgccaagcagattcagcggcagcagatctggcaccgagtacaccctgaccatctccggcgtgcagagagaggacgccgctacctattactgcctgggcggcgtgggcaacgtgtcctacagaaccagcttcggcggaggtactgaggtggtcgtcaaatacggaccgccctgccccccttgccctggccagcctcgcgagccccaggtgtacaccctgcctccctcccaggaagagatgaccaagaaccaggtgtccctgacctgcctggtgaagggcttctaccccagcgacatcgccgtggagtgggagagcaacggccagcctgagaacaactacaagaccacccctcccgtgctggacagcgacggcagcttcttcctgtacagccggctgaccgtggacaagagccggtggcaggaaggcaacgtctttagctgcagcgtgatgcacgaggccctgcacaaccactacacccagaagagcctgagcctgtccctgggcaagatgttctgggtgctggtggtggtgggcggggtgctggcctgctacagcctgctggtgacagtggccttcatcatcttttgggtgaaacggggcagaaagaaactcctgtatatattcaaacaaccatttatgagaccagtacaaactactcaagaggaagatggctgtagctgccgatttccagaagaagaagaaggaggatgtgaactgcgggtgaagttcagcagaagcgccgacgcccctgcctaccagcagggccagaatcagctgtacaacgagctgaacctgggcagaagggaagagtacgacgtcctggataagcggagaggccgggaccctgagatgggcggcaagcctcggcggaagaacccccaggaaggcctgtataacgaactgcagaaagacaagatggccgaggcctacagcgagatcggcatgaagggcgagcggaggcggggcaagggccacgacggcctgtatcagggcctgtccaccgccaccaaggatacctacgacgccctgcacatgcaggccctgcccccaaggctcgagggcggcggagagggcagaggaagtcttctaacatgcggtgacgtggaggagaatcccggccctaggatgcttctcctggtgacaagccttctgctctgtgagttaccacacccagcattcctcctgatcccacgcaaagtgtgtaacggaataggtattggtgaatttaaagactcactctccataaatgctacgaatattaaacacttcaaaaactgcacctccatcagtggcgatctccacatcctgccggtggcatttaggggtgactccttcacacatactcctcctctggatccacaggaactggatattctgaaaaccgtaaaggaaatcacagggtttttgctgattcaggcttggcctgaaaacaggacggacctccatgcctttgagaacctagaaatcatacgcggcaggaccaagcaacatggtcagttttctcttgcagtcgtcagcctgaacataacatccttgggattacgctccctcaaggagataagtgatggagatgtgataatttcaggaaacaaaaatttgtgctatgcaaatacaataaactggaaaaaactgtttgggacctccggtcagaaaaccaaaattataagcaacagaggtgaaaacagctgcaaggccacaggccaggtctgccatgccttgtgctcccccgagggctgctggggcccggagcccagggactgcgtctcttgccggaatgtcagccgaggcagggaatgcgtggacaagtgcaaccttctggagggtgagccaagggagtttgtggagaactctgagtgcatacagtgccacccagagtgcctgcctcaggccatgaacatcacctgcacaggacggggaccagacaactgtatccagtgtgcccactacattgacggcccccactgcgtcaagacctgcccggcaggagtcatgggagaaaacaacaccctggtctggaagtacgcagacgccggccatgtgtgccacctgtgccatccaaactgcacctacggatgcactgggccaggtcttgaaggctgtccaacgaatgggcctaagatcccgtccatcgccactgggatggtgggggccctcctcttgctgctggtggtggccctggggatcggcctcttcatgtgagcggccgctctagacccgggctgcaggaattcgatatcaagcttatcgataatcaacctctggattacaaaatttgtgaaagattgactggtattcttaactatgttgctccttttacgctatgtggatacgctgctttaatgcctttgtatcatgctattgcttcccgtatggctttcattttctcctccttgtataaatcctggttgctgtctctttatgaggagttgtggcccgttgtcaggcaacgtggcgtggtgtgcactgtgtttgctgacgcaacccccactggttggggcattgccaccacctgtcagctcctttccgggactttcgctttccccctccctattgccacggcggaactcatcgccgcctgccttgcccgctgctggacaggggctcggctgttgggcactgacaattccgtggtgttgtcggggaaatcatcgtcctttccttggctgctcgcctgtgttgccacctggattctgcgcgggacgtccttctgctacgtcccttcggccctcaatccagcggaccttccttcccgcggcctgctgccggctctgcggcctcttccgcgtcttcgccttcgccctcagacgagtcggatctccctttgggccgcctccccgcatcgataccgtcgactagccgtacctttaagaccaatgacttacaaggcagctgtagatcttagccactttttaaaagaaaaggggggactggaagggctaattcactcccaaagaagacaagatctgctttttgcctgtactgggtctctctggttagaccagatctgagcctgggagctctctggctaactagggaacccactgcttaagcctcaataaagcttgccttgagtgcttcaagtagtgtgtgcccgtctgttgtgtgactctggtaactagagatccctcagacccttttagtcagtgtggaaaatctctagcagaattcgatatcaagcttatcgataccgtcgacctcgagggggggcccggtacccaattcgccctatagtgagtcgtattacaattcactggccgtcgttttacaacgtcgtgactgggaaaaccctggcgttacccaacttaatcgccttgcagcacatccccctttcgccagctggcgtaatagcgaagaggcccgcaccgatcgcccttcccaacagttgcgcagcctgaatggcgaatggaaattgtaagcgttaatattttgttaaaattcgcgttaaatttttgttaaatcagctcattttttaaccaataggccgaaatcggcaaaatcccttataaatcaaaagaatagaccgagatagggttgagtgttgttccagtttggaacaagagtccactattaaagaacgtggactccaacgtcaaagggcgaaaaaccgtctatcagggcgatggcccactacgtgaaccatcaccctaatcaagttttttggggtcgaggtgccgtaaagcactaaatcggaaccctaaagggagcccccgatttagagcttgacggggaaagccggcgaacgtggcgagaaaggaagggaagaaagcgaaaggagcgggcgctagggcgctggcaagtgtagcggtcacgctgcgcgtaaccaccacacccgccgcgcttaatgcgccgctacagggcgcgtcaggtggcacttttcggggaaatgtgcgcggaacccctatttgtttatttttctaaatacattcaaatatgtatccgctcatgagacaataaccctgataaatgcttcaataatattgaaaaaggaagagtatgagtattcaacatttccgtgtcgcccttattcccttttttgcggcattttgccttcctgtttttgctcacccagaaacgctggtgaaagtaaaagatgctgaagatcagttgggtgcacgagtgggttacatcgaactggatctcaacagcggtaagatccttgagagttttcgccccgaagaacgttttccaatgatgagcacttttaaagttctgctatgtggcgcggtattatcccgtattgacgccgggcaagagcaactcggtcgccgcatacactattctcagaatgacttggttgagtactcaccagtcacagaaaagcatcttacggatggcatgacagtaagagaattatgcagtgctgccataaccatgagtgataacactgcggccaacttacttctgacaacgatcggaggaccgaaggagctaaccgcttttttgcacaacatgggggatcatgtaactcgccttgatcgttgggaaccggagctgaatgaagccataccaaacgacgagcgtgacaccacgatgcctgtagcaatggcaacaacgttgcgcaaactattaactggcgaactacttactctagcttcccggcaacaattaatagactggatggaggcggataaagttgcaggaccacttctgcgctcggcccttccggctggctggtttattgctgataaatctggagccggtgagcgtgggtctcgcggtatcattgcagcactggggccagatggtaagccctcccgtatcgtagttatctacacgacggggagtcaggcaactatggatgaacgaaatagacagatcgctgagataggtgcctcactgattaagcattggtaactgtcagaccaagtttactcatatatactttagattgatttaaaacttcatttttaatttaaaaggatctaggtgaagatcctttttgataatctcatgaccaaaatcccttaacgtgagttttcgttccactgagcgtcagaccccgtagaaaagatcaaaggatcttcttgagatcctttttttctgcgcgtaatctgctgcttgcaaacaaaaaaaccaccgctaccagcggtggtttgtttgccggatcaagagctaccaactctttttccgaaggtaactggcttcagcagagcgcagataccaaatactgttcttctagtgtagccgtagttaggccaccacttcaagaactctgtagcaccgcctacatacctcgctctgctaatcctgttaccagtggctgctgccagtggcgataagtcgtgtcttaccgggttggactcaagacgatagttaccggataaggcgcagcggtcgggctgaacggggggttcgtgcacacagcccagcttggagcgaacgacctacaccgaactgagatacctacagcgtgagctatgagaaagcgccacgcttcccgaagggagaaaggcggacaggtatccggtaagcggcagggtcggaacaggagagcgcacgagggagcttccagggggaaacgcctggtatctttatagtcctgtcgggtttcgccacctctgacttgagcgtcgatttttgtgatgctcgtcaggggggcggagcctatggaaaaacgccagcaacgcggcctttttacggttcctggccttttgctggccttttgctcacatgttctttcctgcgttatcccctgattctgtggataaccgtattaccgcctttgagtgagctgataccgctcgccgcagccgaacgaccgagcgcagcgagtcagtgagcgaggaagcggaagagcgcccaatacgcaaaccgcctctccccgcgcgttggccgattcattaatgcagctggcacgacaggtttcccgactggaaagcgggcagtgagcgcaacgcaattaatgtgagttagctcactcattaggcaccccaggctttacactttatgcttccggctcgtatgttgtgtggaattgtgagcggataacaatttcacacaggaaacagctatgaccatgattacgccaagctcgaaattaaccctcactaaagggaacaaaagctggagctccaccgcggtggcggcctcgaggtcgagatccggtcgaccagcaaccatagtcccgcccctaactccgcccatcccgcccctaactccgcccagttccgcccattctccgccccatggctgactaattttttttatttatgcagaggccgaggccgcctcggcctctgagctattccagaagtagtgaggaggcttttttggaggcctaggcttttgcaaaaagcttcgacggtatcgattggctcatgtccaacattaccgccatgttgacattgattattgactagttattaatagtaatcaattacggggtcattagttcatagcccatatatggagttccgcgttacataacttacggtaaatggcccgcctggctgaccgcccaacgacccccgcccattgacgtcaataatgacgtatgttcccatagtaacgccaatagggactttccattgacgtcaatgggtggagtatttacggtaaactgcccacttggcagtacatcaagtgtatcatatgccaagtacgccccctattgacgtcaatgacggtaaatggcccgcctggcattatgcccagtacatgaccttatgggactttcctacttggcagtacatctacgtattagtcatcgctattaccatggtgatgcggttttggcagtacatcaatgggcgtggatagcggtttgactcacggggatttccaagtctccaccccattgacgtcaatgggagtttgttttggcaccaaaatcaacgggactttccaaaatgtcgtaacaactccgccccattgacgcaaatgggcggtaggcgtgtacggaattcggagtggcgagccctcagatcctgcatataagcagctgctttttgcctgtactgggtctctctg

SEQ ID NO: 48 - protein, 838 aa, synthetic construct
  REGION 1..838: note = Synthetic
MLLLVTSLLLCELPHPAFLLIPQSVKESEGDLVTPAGNLTLTCTASGSDINDYPISWVRQAPGKGLEWIGFINSGGSTWYASWVKGRFTISRTSTTVDLKMTSLTTDDTATYFCARGYSTYYGDFNIWGPGTLVTISSGGGGSGGGGSGGGGSELVMTQTPSSTSGAVGGTVTINCQASQSIDSNLAWFQQKPGQPPTLLIYRASNLASGVPSRFSGSRSGTEYTLTISGVQREDAATYYCLGGVGNVSYRTSFGGGTEVVVKESKYGPPCPPCPMFWVLVVVGGVLACYSLLVTVAFIIFWVKRGRKKLLYIFKQPFMRPVQTTQEEDGCSCRFPEEEEGGCELRVKFSRSADAPAYQQGQNQLYNELNLGRREEYDVLDKRRGRDPEMGGKPRRKNPQEGLYNELQKDKMAEAYSEIGMKGERRRGKGHDGLYQGLSTATKDTYDALHMQALPPRLEGGGEGRGSLLTCGDVEENPGPRMLLLVTSLLLCELPHPAFLLIPRKVCNGIGIGEFKDSLSINATNIKHFKNCTSISGDLHILPVAFRGDSFTHTPPLDPQELDILKTVKEITGFLLIQAWPENRTDLHAFENLEIIRGRTKQHGQFSLAVVSLNITSLGLRSLKEISDGDVIISGNKNLCYANTINWKKLFGTSGQKTKIISNRGENSCKATGQVCHALCSPEGCWGPEPRDCVSCRNVSRGRECVDKCNLLEGEPREFVENSECIQCHPECLPQAMNITCTGRGPDNCIQCAHYIDGPHCVKTCPAGVMGENNTLVWKYADAGHVCHLCHPNCTYGCTGPGLEGCPTNGPKIPSIATGMVGALLLLLVVALGIGLFM

SEQ ID NO: 49 - protein, 119 aa, synthetic construct
  REGION 1..119: note = Synthetic
ESKYGPPCPPCPGQPREPQVYTLPPSQEEMTKNQVSLTCLVKGFYPSDIAVEWESNGQPENNYKTTPPVLDSDGSFFLYSRLTVDKSRWQEGNVFSCSVMHEALHNHYTQKSLSLSLGK

SEQ ID NO: 50 - protein, 229 aa, synthetic construct
  REGION 1..229: note = Synthetic
ESKYGPPCPPCPAPEFLGGPSVFLFPPKPKDTLMISRTPEVTCVVVDVSQEDPEVQFNWYVDGVEVHNAKTKPREEQFNSTYRVVSVLTVLHQDWLNGKEYKCKVSNKGLPSSIEKTISKAKGQPREPQVYTLPPSQEEMTKNQVSLTCLVKGFYPSDIAVEWESNGQPENNYKTTPPVLDSDGSFFLYSRLTVDKSRWQEGNVFSCSVMHEALHNHYTQKSLSLSLGK

SEQ ID NO: 51 - protein, 9 aa, synthetic construct
  REGION 1..9: note = Synthetic
YGPPCPPCP

SEQ ID NO: 52 - protein, 10 aa, synthetic construct
  REGION 1..10: note = Synthetic
KYGPPCPPCP

SEQ ID NO: 53 - protein, 14 aa, synthetic construct
  REGION 1..14: note = Synthetic
EVVVKYGPPCPPCP

SEQ ID NO: 54 - DNA, 2529 bp, synthetic construct
  misc_feature 1..2529: note = Synthetic
  source 1..2529: mol_type = other DNA
atgcttctcctggtgacaagccttctgctctgtgagttaccacacccagcattcctcctgatcccagatatccagatgacccagtccccgagctccctgtccgcctctgtgggcgatagggtcaccatcacctgccgtgccagtcaggatgtgaatactgctgtagcctggtatcaacagaaaccaggaaaagctccgaaactactgatttactcggcatccttcctctactctggagtcccttctcgcttctctggttccagatctgggacggatttcactctgaccatcagcagtctgcagccggaagacttcgcaacttattactgtcagcaacattatactactcctcccacgttcggacagggtaccaaggtggagatcaaaggcagtactagcggcggtggctccgggggcggatccggtgggggcggcagcagcgaggttcagctggtggagtctggcggtggcctggtgcagccagggggctcactccgtttgtcctgtgcagcttctggcttcaacattaaagacacctatatacactgggtgcgtcaggccccgggtaagggcctggaatgggttgcaaggatttatcctacgaatggttatactagatatgccgatagcgtcaagggccgtttcactataagcgcagacacatccaaaaacacagcctacctgcagatgaacagcctgcgtgctgaggacactgccgtctattattgttctagatggggaggggacggcttctatgctatggactactggggtcaaggaaccctggtcaccgtctcgagtgagagcaagtacggaccgccctgccccccttgccctatgttctgggtgctggtggtggtcggaggcgtgctggcctgctacagcctgctggtcaccgtggccttcatcatcttttgggtgaaacggggcagaaagaaactcctgtatatattcaaacaaccatttatgagaccagtacaaactactcaagaggaagatggctgtagctgccgatttccagaagaagaagaaggaggatgtgaactgcgggtgaagttcagcagaagcgccgacgcccctgcctaccagcagggccagaatcagctgtacaacgagctgaacctgggcagaagggaagagtacgacgtcctggataagcggagaggccgggaccctgagatgggcggcaagcctcggcggaagaacccccaggaaggcctgtataacgaactgcagaaagacaagatggccgaggcctacagcgagatcggcatgaagggcgagcggaggcggggcaagggccacgacggcctgtatcagggcctgtccaccgccaccaaggatacctacgacgccctgcacatgcaggccctgcccccaaggctcgagggcggcggagagggcagaggaagtcttctaacatgcggtgacgtggaggagaatcccggccctaggatgcttctcctggtgacaagccttctgctctgtgagttaccacacccagcattcctcctgatcccacgcaaagtgtgtaacggaataggtattggtgaatttaaagactcactctccataaatgctacgaatattaaacacttcaaaaactgcacctccatcagtggcgatctccacatcctgccggtggcatttaggggtgactccttcacacatactcctcctctggatccacaggaactggatattctgaaaaccgtaaaggaaatcacagggtttttgctgattcaggcttggcctgaaaacaggacggacctccatgcctttgagaacctagaaatcatacgcggcaggaccaagcaacatggtcagttttctcttgcagtcgtcagcctgaacataacatccttgggattacgctccctcaaggagataagtgatggagatgtgataatttcaggaaacaaaaatttgtgctatgcaaatacaataaactggaaaaaactgtttgggacctccggtcagaaaaccaaaattataagcaacagaggtgaaaacagctgcaaggccacaggccaggtctgccatgccttgtgctcccccgagggctgctggggcccggagcccagggactgcgtctcttgccggaatgtcagccgaggcagggaatgcgtggacaagtgcaaccttctggagggtgagccaagggagtttgtggagaactctgagtgcatacagtgccacccagagtgcctgcctcaggccatgaacatcacctgcacaggacggggaccagacaactgtatccagtgtgcccactacattgacggcccccactgcgtcaagacctgcccggcaggagtcatgggagaaaacaacaccctggtctggaagtacgcagacgccggccatgtgtgccacctgtgccatccaaactgcacctacggatgcactgggccaggtcttgaaggctgtccaacgaatgggcctaagatcccgtccatcgccactgggatggtgggggccctcctcttgctgctggtggtggccctggggatcggcctcttcatgtga

SEQ ID NO: 55 - DNA, 2850 bp, synthetic construct
  misc_feature 1..2850: note = Synthetic
  source 1..2850: mol_type = other DNA
atgcttctcctggtgacaagccttctgctctgtgagttaccacacccagcattcctcctgatcccagatatccagatgacccagtccccgagctccctgtccgcctctgtgggcgatagggtcaccatcacctgccgtgccagtcaggatgtgaatactgctgtagcctggtatcaacagaaaccaggaaaagctccgaaactactgatttactcggcatccttcctctactctggagtcccttctcgcttctctggttccagatctgggacggatttcactctgaccatcagcagtctgcagccggaagacttcgcaacttattactgtcagcaacattatactactcctcccacgttcggacagggtaccaaggtggagatcaaaggcagtactagcggcggtggctccgggggcggatccggtgggggcggcagcagcgaggttcagctggtggagtctggcggtggcctggtgcagccagggggctcactccgtttgtcctgtgcagcttctggcttcaacattaaagacacctatatacactgggtgcgtcaggccccgggtaagggcctggaatgggttgcaaggatttatcctacgaatggttatactagatatgccgatagcgtcaagggccgtttcactataagcgcagacacatccaaaaacacagcctacctgcagatgaacagcctgcgtgctgaggacactgccgtctattattgttctagatggggaggggacggcttctatgctatggactactggggtcaaggaaccctggtcaccgtctcgagtgagagcaagtacggaccgccctgccccccttgccctggccagcctagagaaccccaggtgtacaccctgcctcccagccaggaagagatgaccaagaaccaggtgtccctgacctgcctggtcaaaggcttctaccccagcgatatcgccgtggaatgggagagcaacggccagcccgagaacaactacaagaccaccccccctgtgctggacagcgacggcagcttcttcctgtactcccggctgaccgtggacaagagccggtggcaggaaggcaacgtcttcagctgcagcgtgatgcacgaggccctgcacaaccactacacccagaagtccctgagcctgagcctgggcaagatgttctgggtgctggtggtggtcggaggcgtgctggcctgctacagcctgctggtcaccgtggccttcatcatcttttgggtgaaacggggcagaaagaaactcctgtatatattcaaacaaccatttatgagaccagtacaaactactcaagaggaagatggctgtagctgccgatttccagaagaagaagaaggaggatgtgaactgcgggtgaagttcagcagaagcgccgacgcccctgcctaccagcagggccagaatcagctgtacaacgagctgaacctgggcagaagggaagagtacgacgtcctggataagcggagaggccgggaccctgagatgggcggcaagcctcggcggaagaacccccaggaaggcctgtataacgaactgcagaaagacaagatggccgaggcctacagcgagatcggcatgaagggcgagcggaggcggggcaagggccacgacggcctgtatcagggcctgtccaccgccaccaaggatacctacgacgccctgcacatgcaggccctgcccccaaggctcgagggcggcggagagggcagaggaagtcttctaacatgcggtgacgtggaggagaatcccggccctaggatgcttctcctggtgacaagccttctgctctgtgagttaccacacccagcattcctcctgatcccacgcaaagtgtgtaacggaataggtattggtgaatttaaagactcactctccataaatgctacgaatattaaacacttcaaaaactgcacctccatcagtggcgatctccacatcctgccggtggcatttaggggtgactccttcacacatactcctcctctggatccacaggaactggatattctgaaaaccgtaaaggaaatcacagggtttttgctgattcaggcttggcctgaaaacaggacggacctccatgcctttgagaacctagaaatcatacgcggcaggaccaagcaacatggtcagttttctcttgcagtcgtcagcctgaacataacatccttgggattacgctccctcaaggagataagtgatggagatgtgataatttcaggaaacaaaaatttgtgctatgcaaatacaataaactggaaaaaactgtttgggacctccggtcagaaaaccaaaattataagcaacagaggtgaaaacagctgcaaggccacaggccaggtctgccatgccttgtgctcccccgagggctgctggggcccggagcccagggactgcgtctcttgccggaatgtcagccgaggcagggaatgcgtggacaagtgcaaccttctggagggtgagccaagggagtttgtggagaactctgagtgcatacagtgccacccagagtgcctgcctcaggccatgaacatcacctgcacaggacggggaccagacaactgtatccagtgtgcccactacattgacggcccccactgcgtcaagacctgcccggcaggagtcatgggagaaaacaacaccctggtctggaagtacgcagacgccggccatgtgtgccacctgtgccatccaaactgcacctacggatgcactgggccaggtcttgaaggctgtccaacgaatgggcctaagatcccgtccatcgccactgggatggtgggggccctcctcttgctgctggtggtggccctggggatcggcctcttcatgtga

SEQ ID NO: 56 - DNA, 3180 bp, synthetic construct
  misc_feature 1..3180: note = Synthetic
  source 1..3180: mol_type = other DNA
atgcttctcctggtgacaagccttctgctctgtgagttaccacacccagcattcctcctgatcccagatatccagatgacccagtccccgagctccctgtccgcctctgtgggcgatagggtcaccatcacctgccgtgccagtcaggatgtgaatactgctgtagcctggtatcaacagaaaccaggaaaagctccgaaactactgatttactcggcatccttcctctactctggagtcccttctcgcttctctggttccagatctgggacggatttcactctgaccatcagcagtctgcagccggaagacttcgcaacttattactgtcagcaacattatactactcctcccacgttcggacagggtaccaaggtggagatcaaaggcagtactagcggcggtggctccgggggcggatccggtgggggcggcagcagcgaggttcagctggtggagtctggcggtggcctggtgcagccagggggctcactccgtttgtcctgtgcagcttctggcttcaacattaaagacacctatatacactgggtgcgtcaggccccgggtaagggcctggaatgggttgcaaggatttatcctacgaatggttatactagatatgccgatagcgtcaagggccgtttcactataagcgcagacacatccaaaaacacagcctacctgcagatgaacagcctgcgtgctgaggacactgccgtctattattgttctagatggggaggggacggcttctatgctatggactactggggtcaaggaaccctggtcaccgtctcgagtgagagcaagtacggaccgccctgccccccttgccctgcccccgagttcctgggcggacccagcgtgttcctgttcccccccaagcccaaggacaccctgatgatcagccggacccccgaggtgacctgcgtggtggtggacgtgagccaggaagatcccgaggtccagttcaattggtacgtggacggcgtggaagtgcacaacgccaagaccaagcccagagaggaacagttcaacagcacctaccgggtggtgtctgtgctgaccgtgctgcaccaggactggctgaacggcaaagaatacaagtgcaaggtgtccaacaagggcctgcccagcagcatcgaaaagaccatcagcaaggccaagggccagcctcgcgagccccaggtgtacaccctgcctccctcccaggaagagatgaccaagaaccaggtgtccctgacctgcctggtgaagggcttctaccccagcgacatcgccgtggagtgggagagcaacggccagcctgagaacaactacaagaccacccctcccgtgctggacagcgacggcagcttcttcctgtacagccggctgaccgtggacaagagccggtggcaggaaggcaacgtctttagctgcagcgtgatgcacgaggccctgcacaaccactacacccagaagagcctgagcctgtccctgggcaagatgttctgggtgctggtggtggtgggcggggtgctggcctgctacagcctgctggtgacagtggccttcatcatcttttgggtgaaacggggcagaaagaaactcctgtatatattcaaacaaccatttatgagaccagtacaaactactcaagaggaagatggctgtagctgccgatttccagaagaagaagaaggaggatgtgaactgcgggtgaagttcagcagaagcgccgacgcccctgcctaccagcagggccagaatcagctgtacaacgagctgaacctgggcagaagggaagagtacgacgtcctggataagcggagaggccgggaccctgagatgggcggcaagcctcggcggaagaacccccaggaaggcctgtataacgaactgcagaaagacaagatggccgaggcctacagcgagatcggcatgaagggcgagcggaggcggggcaagggccacgacggcctgtatcagggcctgtccaccgccaccaaggatacctacgacgccctgcacatgcaggccctgcccccaaggctcgagggcggcggagagggcagaggaagtcttctaacatgcggtgacgtggaggagaatcccggccctaggatgcttctcctggtgacaagccttctgctctgtgagttaccacacccagcattcctcctgatcccacgcaaagtgtgtaacggaataggtattggtgaatttaaagactcactctccataaatgctacgaatattaaacacttcaaaaactgcacctccatcagtggcgatctccacatcctgccggtggcatttaggggtgactccttcacacatactcctcctctggatccacaggaactggatattctgaaaaccgtaaaggaaatcacagggtttttgctgattcaggcttggcctgaaaacaggacggacctccatgcctttgagaacctagaaatcatacgcggcaggaccaagcaacatggtcagttttctcttgcagtcgtcagcctgaacataacatccttgggattacgctccctcaaggagataagtgatggagatgtgataatttcaggaaacaaaaatttgtgctatgcaaatacaataaactggaaaaaactgtttgggacctccggtcagaaaaccaaaattataagcaacagaggtgaaaacagctgcaaggccacaggccaggtctgccatgccttgtgctcccccgagggctgctggggcccggagcccagggactgcgtctcttgccggaatgtcagccgaggcagggaatgcgtggacaagtgcaaccttctggagggtgagccaagggagtttgtggagaactctgagtgcatacagtgccacccagagtgcctgcctcaggccatgaacatcacctgcacaggacggggaccagacaactgtatccagtgtgcccactacattgacggcccccactgcgtcaagacctgcccggcaggagtcatgggagaaaacaacaccctggtctggaagtacgcagacgccggccatgtgtgccacctgtgccatccaaactgcacctacggatgcactgggccaggtcttgaaggctgtccaacgaatgggcctaagatcccgtccatcgccactgggatggtgggggccctcctcttgctgctggtggtggccctggggatcggcctcttcatgtga

SEQ ID NO: 57 - protein, 11 aa, synthetic construct
RASQDISKYLN

SEQ ID NO: 58 - protein, 7 aa, synthetic construct
SRLHSGV

SEQ ID NO: 59 - protein, 9 aa, synthetic construct
GNTLPYTFG

SEQ ID NO: 60 - protein, 5 aa, synthetic construct
DYGVS

SEQ ID NO: 61 - protein, 16 aa, synthetic construct
VIWGSETTYYNSALKS

SEQ ID NO: 62 - protein, 7 aa, synthetic construct
YAMDYWG

SEQ ID NO: 63 - protein, 11 aa, synthetic construct
ASGFDFSAYYM

SEQ ID NO: 64 - protein, 7 aa, synthetic construct
TIYPSSG

SEQ ID NO: 65 - protein, 9 aa, synthetic construct
ADRATYFCA

SEQ ID NO: 66 - protein, 6 aa, synthetic construct
DTIDWY

SEQ ID NO: 67 - protein, 16 aa, synthetic construct
VQSDGSYTKRPGVPDR

SEQ ID NO: 68 - protein, 8 aa, synthetic construct
YIGGYVFG

SEQ ID NO: 69 - protein, 11 aa, synthetic construct
SGSDINDYPIS

SEQ ID NO: 70 - protein, 7 aa, synthetic construct
INSGGST

SEQ ID NO: 71 - protein, 8 aa, synthetic construct
YFCARGYS

SEQ ID NO: 72 - protein, 5 aa, synthetic construct
SNLAW

SEQ ID NO: 73 - protein, 16 aa, synthetic construct
RASNLASGVPSRFSGS

SEQ ID NO: 74 - protein, 8 aa, synthetic construct
NVSYRTSF

SEQ ID NO: 75 - DNA, 2911 bp, synthetic construct
  source 1..2911: mol_type = other DNA
gttagaccagatctgagcctgggagctctctggctaactagggaacccactgcttaagcctcaataaagcttgccttgagtgcttcaagtagtgtgtgcccgtctgttgtgtgactctggtaactagagatccctcagacccttttagtcagtgtggaaaatctctagcagtggcgcccgaacagggacttgaaagcgaaagggaaaccagaggagctctctcgacgcaggactcggcttgctgaagcgcgcacggcaagaggcgaggggcggcgactggtgagtacgccaaaaattttgactagcggaggctagaaggagagagatgggtgcgagagcgtcagtattaagcgggggagaattagatcgatgggaaaaaattcggttaaggccagggggaaagaaaaaatataaattaaaacatatagtatgggcaagcagggagctagaacgattcgcagttaatcctggcctgttagaaacatcagaaggctgtagacaaatactgggacagctacaaccatcccttcagacaggatcagaagaacttagatcattatataatacagtagcaaccctctattgtgtgcatcaaaggatagagataaaagacaccaaggaagctttagacaagatagaggaagagcaaaacaaaagtaagaaaaaagcacagcaagcagcagctgacacaggacacagcaatcaggtcagccaaaattaccctatagtgcagaacatccaggggcaaatggtacatcaggccatatcacctagaactttaaatgcatgggtaaaagtagtagaagagaaggctttcagcccagaagtgatacccatgttttcagcattatcagaaggagccaccccacaagatttaaacaccatgctaaacacagtggggggacatcaagcagccatgcaaatgttaaaagagaccatcaatgaggaagctgcaggcaaagagaagagtggtgcagagagaaaaaagagcagtgggaataggagctttgttccttgggttcttgggagcagcaggaagcactatgggcgcagcgtcaatgacgctgacggtacaggccagacaattattgtctggtatagtgcagcagcagaacaatttgctgagggctattgaggcgcaacagcatctgttgcaactcacagtctggggcatcaagcagctccaggcaagaatcctggctgtggaaagatacctaaaggatcaacagctcctggggatttggggttgctctggaaaactcatttgcaccactgctgtgccttggatctacaaatggcagtattcatccacaattttaaaagaaaaggggggattggggggtacagtgcaggggaaagaatagtagacataatagcaacagacatacaaactaaagaattacaaaaacaaattacaaaaattcaaaattttcgggtttattacagggacagcagagatccagtttggggatcaattgcatgaagaatctgcttagggttaggcgttttgcgctgcttcgcgaggatctgcgatcgctccggtgcccgtcagtgggcagagcgcacatcgcccacagtccccgagaagttggggggaggggtcggcaattgaaccggtgcctagagaaggtggcgcggggtaaactgggaaagtgatgtcgtgtactggctccgcctttttcccgagggtgggggagaaccgtatataagtgcagtagtcgccgtgaacgttctttttcgcaacgggtttgccgccagaacacagctgaagcttcgaggggctcgcatctctccttcacgcgcccgccgccctacctgaggccgccatccacgccggttgagtcgcgttctgccgcctcccgcctgtggtgcctcctgaactgcgtccgccgtctaggtaagtttaaagctcaggtcgagaccgggcctttgtccggcgctcccttggagcctacctagactcagccggctctccacgctttgcctgaccctgcttgctcaactctacgtctttgtttcgttttctgttctgcgccgttacagatccaagctgtgaccggcgcctacggctagcgaattcctcgaggccaccatgctgctgctggtgacaagcctgctgctgtgcgagctgccccaccccgcctttctgctgatcccccaggaacagctcgtcgaaagcggcggcagactggtgacacctggcggcagcctgaccctgagctgcaaggccagcggcttcgacttcagcgcctactacatgagctgggtccgccaggcccctggcaagggactggaatggatcgccaccatctaccccagcagcggcaagacctactacgccacctgggtgaacggacggttcaccatctccagcgacaacgcccagaacaccgtggacctgcagatgaacagcctgacagccgccgaccgggccacctacttttgcgccagagacagctacgccgacgacggcgccctgttcaacatctggggccctggcaccctggtgacaatctctagcggcggaggcggatctggtggcggaggaagtggcggcggaggatctgagctggtgctgacccagagcccctctgtgtctgctgccctgggaagccctgccaagatcacctgtaccctgagcagcgcccacaagaccgacaccatcgactggtatcagcagctgcagggcgaggcccccagatacctgatgcaggtgcagagcgacggcagctacaccaagaggccaggcgtgcccgaccggttcagcggatctagctctggcgccgaccgctacctgatcatccccagcgtgcaggccgatgacgaggccgattactactgtggcgccgactacatcggcggctacgtgttcggcggaggcacccagctgaccgtgaccggcgagtctaag

SEQ ID NO: 76 - DNA, 27 bp, synthetic construct
  source 1..27: mol_type = other DNA
tacggaccgccctgccccccttgccct

SEQ ID NO: 77 - DNA, 330 bp, synthetic construct
  source 1..330: mol_type = other DNA
gcccccgagttcctgggcggacccagcgtgttcctgttcccccccaagcccaaggacaccctgatgatcagccggacccccgaggtgacctgcgtggtggtggacgtgagccaggaagatcccgaggtccagttcaattggtacgtggacggcgtggaagtgcacaacgccaagaccaagcccagagaggaacagttcaacagcacctaccgggtggtgtctgtgctgaccgtgctgcaccaggactggctgaacggcaaagaatacaagtgcaaggtgtccaacaagggcctgcccagcagcatcgaaaagaccatcagcaaggccaag

SEQ ID NO: 78 - DNA, 321 bp, synthetic construct
  source 1..321: mol_type = other DNA
ggccagcctcgcgagccccaggtgtacaccctgcctccctcccaggaagagatgaccaagaaccaggtgtccctgacctgcctggtgaagggcttctaccccagcgacatcgccgtggagtgggagagcaacggccagcctgagaacaactacaagaccacccctcccgtgctggacagcgacggcagcttcttcctgtacagccggctgaccgtggacaagagccggtggcaggaaggcaacgtctttagctgcagcgtgatgcacgaggccctgcacaaccactacacccagaagagcctgagcctgtccctgggcaag

SEQ ID NO: 79 - DNA, 210 bp, synthetic construct
  source 1..210: mol_type = other DNA
atgttctgggtgctggtggtggtgggcggggtgctggcctgctacagcctgctggtgacagtggccttcatcatcttttgggtgaaacggggcagaaagaaactcctgtatatattcaaacaaccatttatgagaccagtacaaactactcaagaggaagatggctgtagctgccgatttccagaagaagaagaaggaggatgtgaactg

SEQ ID NO: 80 - DNA, 336 bp, synthetic construct; identical to SEQ ID NO: 7
  source 1..336: mol_type = other DNA

SEQ ID NO: 81 - DNA, 72 bp, synthetic construct; identical to SEQ ID NO: 8
  source 1..72: mol_type = other DNA

SEQ ID NO: 82 - DNA, 5844 bp, synthetic construct
  source 1..5844: mol_type = other DNA
atgcttctcctggtgacaagccttctgctctgtgagttaccacacccagcattcctcctgatcccacgcaaagtgtgtaacggaataggtattggtgaatttaaagactcactctccataaatgctacgaatattaaacacttcaaaaactgcacctccatcagtggcgatctccacatcctgccggtggcatttaggggtgactccttcacacatactcctcctctggatccacaggaactggatattctgaaaaccgtaaaggaaatcacagggtttttgctgattcaggcttggcctgaaaacaggacggacctccatgcctttgagaacctagaaatcatacgcggcaggaccaagcaacatggtcagttttctcttgcagtcgtcagcctgaacataacatccttgggattacgctccctcaaggagataagtgatggagatgtgataatttcaggaaacaaaaatttgtgctatgcaaatacaataaactggaaaaaactgtttgggacctccggtcagaaaaccaaaattataagcaacagaggtgaaaacagctgcaaggccacaggccaggtctgccatgccttgtgctcccccgagggctgctggggcccggagcccagggactgcgtctcttgccggaatgtcagccgaggcagggaatgcgtggacaagtgcaaccttctggagggtgagccaagggagtttgtggagaactctgagtgcatacagtgccacccagagtgcctgcctcaggccatgaacatcacctgcacaggacggggaccagacaactgtatccagtgtgcccactacattgacggcccccactgcgtcaagacctgcccggcaggagtcatgggagaaaacaacaccctggtctggaagtacgcagacgccggccatgtgtgccacctgtgccatccaaactgcacctacggatgcactgggccaggtcttgaaggctgtccaacgaatgggcctaagatcccgtccatcgccactgggatggtgggggccctcctcttgctgctggtggtggccctggggatcggcctcttcatgtgagcggccgctctagacccgggctgcaggaattcgatatcaagcttatcgataatcaacctctggattacaaaatttgtgaaagattgactggtattcttaactatgttgctccttttacgctatgtggatacgctgctttaatgcctttgtatcatgctattgcttcccgtatggctttcattttctcctccttgtataaatcctggttgctgtctctttatgaggagttgtggcccgttgtcaggcaacgtggcgtggtgtgcactgtgtttgctgacgcaacccccactggttggggcattgccaccacctgtcagctcctttccgggactttcgctttccccctccctattgccacggcggaactcatcgccgcctgccttgcccgctgctggacaggggctcggctgttgggcactgacaattccgtggtgttgtcggggaaatcatcgtcctttccttggctgctcgcctgtgttgccacctggattctgcgcgggacgtccttctgctacgtcccttcggccctcaatccagcggaccttccttcccgcggcctgctgccggctctgcggcctcttccgcgtcttcgccttcgccctcagacgagtcggatctccctttgggccgcctccccgcatcgataccgtcgactagccgtacctttaagaccaatgacttacaaggcagctgtagatcttagccactttttaaaagaaaaggggggactggaagggctaattcactcccaaagaagacaagatctgctttttgcctgtactgggtctctctggttagaccagatctgagcctgggagctctctggctaactagggaacccactgcttaagcctcaataaagcttgccttgagtgcttcaagtagtgtgtgcccgtctgttgtgtgactctggtaactagagatccctcagacccttttagtcagtgtggaaaatctctagcagaattcgatatcaagcttatcgataccgtcgacctcgagggggggcccggtacccaattcgccctatagtgagtcgtattacaattcactggccgtcgttttacaacgtcgtgactgggaaaaccctggcgttacccaacttaatcgccttgcagcacatccccctttcgccagctggcgtaatagcgaagaggcccgcaccgatcgcccttcccaacagttgcgcagcctgaatggcgaatggaaattgtaagcgttaatattttgttaaaattcgcgttaaatttttgttaaatcagctcattttttaaccaataggccgaaatcggcaaaatcccttataaatcaaaagaatagaccgagatagggttgagtgttgttccagtttggaacaagagtccactattaaagaacgtggactccaacgtcaaagggcgaaaaaccgtctatcagggcgatggcccactacgtgaaccatcaccctaatcaagttttttggggtcgaggtgccgtaaagcactaaatcggaaccctaaagggagcccccgatttagagcttgacggggaaagccggcgaacgtggcgagaaaggaagggaagaaagcgaaaggagcgggcgctagggcgctggcaagtgtagcggtcacgctgcgcgtaaccaccacacccgccgcgcttaatgcgccgctacagggcgcgtcaggtggcacttttcggggaaatgtgcgcggaacccctatttgtttatttttctaaatacattcaaatatgtatccgctcatgagacaataaccctgataaatgcttcaataatattgaaaaaggaagagtatgagtattcaacatttccgtgtcgcccttattcccttttttgcggcattttgccttcctgtttttgctcacccagaaacgctggtgaaagtaaaagatgctgaagatcagttgggtgcacgagtgggttacatcgaactggatctcaacagcggtaagatccttgagagttttcgccccgaagaacgttttccaatgatgagcacttttaaagttctgctatgtggcgcggtattatcccgtattgacgccgggcaagagcaactcggtcgccgcatacactattctcagaatgacttggttgagtactcaccagtcacagaaaagcatcttacggatggcatgacagtaagagaattatgcagtgctgccataaccatgagtgataacactgcggccaacttacttctgacaacgatcggaggaccgaaggagctaaccgcttttttgcacaacatgggggatcatgtaactcgccttgatcgttgggaaccggagctgaatgaagccataccaaacgacgagcgtgacaccacgatgcctgtagcaatggcaacaacgttgcgcaaactattaactggcgaactacttactctagcttcccggcaacaattaatagactggatggaggcggataaagttgcaggaccacttctgcgctcggcccttccggctggctggtttattgctgataaatctggagccggtgagcgtgggtctcgcggtatcattgcagcactggggccagatggtaagccctcccgtatcgtagttatctacacgacggggagtcaggcaactatggatgaacgaaatagacagatcgctgagataggtgcctcactgattaagcattggtaactgtcagaccaagtttactcatatatactttagattgatttaaaacttcatttttaatttaaaaggatctaggtgaagatcctttttgataatctcatgaccaaaatcccttaacgtgagttttcgttccactgagcgtcagaccccgtagaaaagatcaaaggatcttcttgagatcctttttttctgcgcgtaatctgctgcttgcaaacaaaaaaaccaccgctaccagcggtggtttgtttgccggatcaagagctaccaactctttttccgaaggtaactggcttcagcagagcgcagataccaaatactgttcttctagtgtagccgtagttaggccaccacttcaagaactctgtagcaccgcctacatacctcgctctgctaatcctgttaccagtggctgctgccagtggcgataagtcgtgtcttaccgggttggactcaagacgatagttaccggataaggcgcagcggtcgggctgaacggggggttcgtgcacacagcccagcttggagcgaacgacctacaccgaactgagatacctacagcgtgagctatgagaaagcgccacgcttcccgaagggagaaaggcggacaggtatccggtaagcggcagggtcggaacaggagagcgcacgagggagcttccagggggaaacgcctggtatctttatagtcctgtcgggtttcgccacctctgacttgagcgtcgatttttgtgatgctcgtcaggggggcggagcctatggaaaaacgccagcaacgcggcctttttacggttcctggccttttgctggccttttgctcacatgttctttcctgcgttatcccctgattctgtggataaccgtattaccgcctttgagtgagctgataccgctcgccgcagccgaacgaccgagcgcagcgagtcagtgagcgaggaagcggaagagcgcccaatacgcaaaccgcctctccccgcgcgttggccgattcattaatgcagctggcacgacaggtttcccgactggaaagcgggcagtgagcgcaacgcaattaatgtgagttagctcactcattaggcaccccaggctttacactttatgcttccggctcgtatgttgtgtggaattgtgagcggataacaatttcacacaggaaacagctatgaccatgattacgccaagctcgaaattaaccctcactaaagggaacaaaagctggagctccaccgcggtggcggcctcgaggtcgagatccggtcgaccagcaaccatagtcccgcccctaactccgcccatcccgcccctaactccgcccagttccgcccattctccgccccatggctgactaattttttttatttatgcagaggccgaggccgcctcggcctctgagctattccagaagtagtgaggaggcttttttggaggcctaggcttttgcaaaaagcttcgacggtatcgattggctcatgtccaacattaccgccatgttgacattgattattgactagttattaatagtaatcaattacggggtcattagttcatagcccatatatggagttccgcgttacataacttacggtaaatggcccgcctggctgaccgcccaacgacccccgcccattgacgtcaataatgacgtatgttcccatagtaacgccaatagggactttccattgacgtcaatgggtggagtatttacggtaaactgcccacttggcagtacatcaagtgtatcatatgccaagtacgccccctattgacgtcaatgacggtaaatggcccgcctggcattatgcccagtacatgaccttatgggactttcctacttggcagtacatctacgtattagtcatcgctattaccatggtgatgcggttttggcagtacatcaatgggcgtggatagcggtttgactcacggggatttccaagtctccaccccattgacgtcaatgggagtttgttttggcaccaaaatcaacgggactttccaaaatgtcgtaacaactccgccccattgacgcaaatgggcggtaggcgtgtacggaattcggagtggcgagccctcagatcctgcatataagcagctgctttttgcctgtactgggtctctctg

SEQ ID NO: 83 - protein, 22 aa, synthetic construct
MLLLVTSLLLCELPHPAFLLIP

SEQ ID NO: 84 - protein, 248 aa, synthetic construct
QEQLVESGGRLVTPGGSLTLSCKASGFDFSAYYMSWVRQAPGKGLEWIATIYPSSGKTYYATWVNGRFTISSDNAQNTVDLQMNSLTAADRATYFCARDSYADDGALFNIWGPGTLVTISSGGGGSGGGGSGGGGSELVLTQSPSVSAALGSPAKITCTLSSAHKTDTIDWYQQLQGEAPRYLMQVQSDGSYTKRPGVPDRFSGSSSGADRYLIIPSVQADDEADYYCGADYIGGYVFGGGTQLTVTG

SEQ ID NO: 85 - protein, 12 aa, synthetic construct
ESKYGPPCPPCP

SEQ ID NO: 86 - protein, 110 aa, synthetic construct
APEFLGGPSVFLFPPKPKDTLMISRTPEVTCVVVDVSQEDPEVQFNWYVDGVEVHNAKTKPREEQFNSTYRVVSVLTVLHQDWLNGKEYKCKVSNKGLPSSIEKTISKAK

SEQ ID NO: 87 - protein, 107 aa, synthetic construct
GQPREPQVYTLPPSQEEMTKNQVSLTCLVKGFYPSDIAVEWESNGQPENNYKTTPPVLDSDGSFFLYSRLTVDKSRWQEGNVFSCSVMHEALHNHYTQKSLSLSLGK

SEQ ID NO: 88 - protein, 28 aa, synthetic construct
MFWVLVVVGGVLACYSLLVTVAFIIFWV

SEQ ID NO: 89 - protein, 42 aa, synthetic construct
KRGRKKLLYIFKQPFMRPVQTTQEEDGCSCRFPEEEEGGCEL

SEQ ID NO: 90 - protein, 112 aa, synthetic construct
RVKFSRSADAPAYQQGQNQLYNELNLGRREEYDVLDKRRGRDPEMGGKPRRKNPQEGLYNELQKDKMAEAYSEIGMKGERRRGKGHDGLYQGLSTATKDTYDALHMQALPPR

SEQ ID NO: 91 - protein, 24 aa, synthetic construct
LEGGGEGRGSLLTCGDVEENPGPR

SEQ ID NO: 92 - protein, 357 aa, synthetic construct
MLLLVTSLLLCELPHPAFLLIPRKVCNGIGIGEFKDSLSINATNIKHFKNCTSISGDLHILPVAFRGDSFTHTPPLDPQELDILKTVKEITGFLLIQAWPENRTDLHAFENLEIIRGRTKQHGQFSLAVVSLNITSLGLRSLKEISDGDVIISGNKNLCYANTINWKKLFGTSGQKTKIISNRGENSCKATGQVCHALCSPEGCWGPEPRDCVSCRNVSRGRECVDKCNLLEGEPREFVENSECIQCHPECLPQAMNITCTGRGPDNCIQCAHYIDGPHCVKTCPAGVMGENNTLVWKYADAGHVCHLCHPNCTYGCTGPGLEGCPTNGPKIPSIATGMVGALLLLLVVALGIGLFM

SEQ ID NO: 93 - DNA, 2089 bp, synthetic construct
  source 1..2089: mol_type = other DNA
gttagaccagatctgagcctgggagctctctggctaactagggaacccactgcttaagcctcaataaagcttgccttgagtgcttcaagtagtgtgtgcccgtctgttgtgtgactctggtaactagagatccctcagacccttttagtcagtgtggaaaatctctagcagtggcgcccgaacagggacttgaaagcgaaagggaaaccagaggagctctctcgacgcaggactcggcttgctgaagcgcgcacggcaagaggcgaggggcggcgactggtgagtacgccaaaaattttgactagcggaggctagaaggagagagatgggtgcgagagcgtcagtattaagcgggggagaattagatcgatgggaaaaaattcggttaaggccagggggaaagaaaaaatataaattaaaacatatagtatgggcaagcagggagctagaacgattcgcagttaatcctggcctgttagaaacatcagaaggctgtagacaaatactgggacagctacaaccatcccttcagacaggatcagaagaacttagatcattatataatacagtagcaaccctctattgtgtgcatcaaaggatagagataaaagacaccaaggaagctttagacaagatagaggaagagcaaaacaaaagtaagaaaaaagcacagcaagcagcagctgacacaggacacagcaatcaggtcagccaaaattaccctatagtgcagaacatccaggggcaaatggtacatcaggccatatcacctagaactttaaatgcatgggtaaaagtagtagaagagaaggctttcagcccagaagtgatacccatgttttcagcattatcagaaggagccaccccacaagatttaaacaccatgctaaacacagtggggggacatcaagcagccatgcaaatgttaaaagagaccatcaatgaggaagctgcaggcaaagagaagagtggtgcagagagaaaaaagagcagtgggaataggagctttgttccttgggttcttgggagcagcaggaagcactatgggcgcagcgtcaatgacgctgacggtacaggccagacaattattgtctggtatagtgcagcagcagaacaatttgctgagggctattgaggcgcaacagcatctgttgcaactcacagtctggggcatcaagcagctccaggcaagaatcctggctgtggaaagatacctaaaggatcaacagctcctggggatttggggttgctctggaaaactcatttgcaccactgctgtgccttggatctacaaatggcagtattcatccacaattttaaaagaaaaggggggattggggggtacagtgcaggggaaagaatagtagacataatagcaacagacatacaaactaaagaattacaaaaacaaattacaaaaattcaaaattttcgggtttattacagggacagcagagatccagtttggggatcaattgcatgaagaatctgcttagggttaggcgttttgcgctgcttcgcgaggatctgcgatcgctccggtgcccgtcagtgggcagagcgcacatcgcccacagtccccgagaagttggggggaggggtcggcaattgaaccggtgcctagagaaggtggcgcggggtaaactgggaaagtgatgtcgtgtactggctccgcctttttcccgagggtgggggagaaccgtatataagtgcagtagtcgccgtgaacgttctttttcgcaacgggtttgccgccagaacacagctgaagcttcgaggggctcgcatctctccttcacgcgcccgccgccctacctgaggccgccatccacgccggttgagtcgcgttctgccgcctcccgcctgtggtgcctcctgaactgcgtccgccgtctaggtaagtttaaagctcaggtcgagaccgggcctttgtccggcgctcccttggagcctacctagactcagccggctctccacgctttgcctgaccctgcttgctcaactctacgtctttgtttcgttttctgttctgcgccgttacagatccaagctgtgaccggcgcctacggctagcgaattcctcgaggcc

SEQ ID NO: 94 - DNA, 822 bp, synthetic construct
  source 1..822: mol_type = other DNA
accatgctgctgctggtgacaagcctgctgctgtgcgagctgccccaccccgcctttctgctgatcccccaggaacagctcgtcgaaagcggcggcagactggtgacacctggcggcagcctgaccctgagctgcaaggccagcggcttcgacttcagcgcctactacatgagctgggtccgccaggcccctggcaagggactggaatggatcgccaccatctaccccagcagcggcaagacctactacgccacctgggtgaacggacggttcaccatctccagcgacaacgcccagaacaccgtggacctgcagatgaacagcctgacagccgccgaccgggccacctacttttgcgccagagacagctacgccgacgacggcgccctgttcaacatctggggccctggcaccctggtgacaatctctagcggcggaggcggatctggtggcggaggaagtggcggcggaggatctgagctggtgctgacccagagcccctctgtgtctgctgccctgggaagccctgccaagatcacctgtaccctgagcagcgcccacaagaccgacaccatcgactggtatcagcagctgcagggcgaggcccccagatacctgatgcaggtgcagagcgacggcagctacaccaagaggccaggcgtgcccgaccggttcagcggatctagctctggcgccgaccgctacctgatcatccccagcgtgcaggccgatgacgaggccgattactactgtggcgccgactacatcggcggctacgtgttcggcggaggcacccagctgaccgtgaccggcgagtctaag

SEQ ID NO: 95 - DNA, 2074 bp, synthetic construct
  source 1..2074: mol_type = other DNA
  unsure 2074
gttagaccagatctgagcctgggagctctctggctaactagggaacccactgcttaagcctcaataaagcttgccttgagtgcttcaagtagtgtgtgcccgtctgttgtgtgactctggtaactagagatccctcagacccttttagtcagtgtggaaaatctctagcagtggcgcccgaacagggacttgaaagcgaaagggaaaccagaggagctctctcgacgcaggactcggcttgctgaagcgcgcacggcaagaggcgaggggcggcgactggtgagtacgccaaaaattttgactagcggaggctagaaggagagagatgggtgcgagagcgtcagtattaagcgggggagaattagatcgatgggaaaaaattcggttaaggccagggggaaagaaaaaatataaattaaaacatatagtatgggcaagcagggagctagaacgattcgcagttaatcctggcctgttagaaacatcagaaggctgtagacaaatactgggacagctacaaccatcccttcagacaggatcagaagaacttagatcattatataatacagtagcaaccctctattgtgtgcatcaaaggatagagataaaagacaccaaggaagctttagacaagatagaggaagagcaaaacaaaagtaagaaaaaagcacagcaagcagcagctgacacaggacacagcaatcaggtcagccaaaattaccctatagtgcagaacatccaggggcaaatggtacatcaggccatatcacctagaactttaaatgcatgggtaaaagtagtagaagagaaggctttcagcccagaagtgatacccatgttttcagcattatcagaaggagccaccccacaagatttaaacaccatgctaaacacagtggggggacatcaagcagccatgcaaatgttaaaagagaccatcaatgaggaagctgcaggcaaagagaagagtggtgcagagagaaaaaagagcagtgggaataggagctttgttccttgggttcttgggagcagcaggaagcactatgggcgcagcgtcaatgacgctgacggtacaggccagacaattattgtctggtatagtgcagcagcagaacaatttgctgagggctattgaggcgcaacagcatctgttgcaactcacagtctggggcatcaagcagctccaggcaagaatcctggctgtggaaagatacctaaaggatcaacagctcctggggatttggggttgctctggaaaactcatttgcaccactgctgtgccttggatctacaaatggcagtattcatccacaattttaaaagaaaaggggggattggggggtacagtgcaggggaaagaatagtagacataatagcaacagacatacaaactaaagaattacaaaaacaaattacaaaaattcaaaattttcgggtttattacagggacagcagagatccagtttggggatcaattgcatgaagaatctgcttagggttaggcgttttgcgctgcttcgcgaggatctgcgatcgctccggtgcccgtcagtgggcagagcgcacatcgcccacagtccccgagaagttggggggaggggtcggcaattgaaccggtgcctagagaaggtggcgcggggtaaactgggaaagtgatgtcgtgtactggctccgcctttttcccgagggtgggggagaaccgtatataagtgcagtagtcgccgtgaacgttctttttcgcaacgggtttgccgccagaacacagctgaagcttcgaggggctcgcatctctccttcacgcgcccgccgccctacctgaggccgccatccacgccggttgagtcgcgttctgccgcctcccgcctgtggtgcctcctgaactgcgtccgccgtctaggtaagtttaaagctcaggtcgagaccgggcctttgtccggcgctcccttggagcctacctagactcagccggctctccacgctttgcctgaccctgcttgctcaactctacgtctttgtttcgttttctgttctgcgccgttacagatccaagctgtgaccggcgcctacggctagn

SEQ ID NO: 96 - DNA, 2074 bp, synthetic construct
  source 1..2074: mol_type = other DNA
gttagaccagatctgagcctgggagctctctggctaactagggaacccactgcttaagcctcaataaagcttgccttgagtgcttcaagtagtgtgtgcccgtctgttgtgtgactctggtaactagagatccctcagacccttttagtcagtgtggaaaatctctagcagtggcgcccgaacagggacttgaaagcgaaagggaaaccagaggagctctctcgacgcaggactcggcttgctgaagcgcgcacggcaagaggcgaggggcggcgactggtgagtacgccaaaaattttgactagcggaggctagaaggagagagatgggtgcgagagcgtcagtattaagcgggggagaattagatcgatgggaaaaaattcggttaaggccagggggaaagaaaaaatataaattaaaacatatagtatgggcaagcagggagctagaacgattcgcagttaatcctggcctgttagaaacatcagaaggctgtagacaaatactgggacagctacaaccatcccttcagacaggatcagaagaacttagatcattatataatacagtagcaaccctctattgtgtgcatcaaaggatagagataaaagacaccaaggaagctttagacaagatagaggaagagcaaaacaaaagtaagaaaaaagcacagcaagcagcagctgacacaggacacagcaatcaggtcagccaaaattaccctatagtgcagaacatccaggggcaaatggtacatcaggccatatcacctagaactttaaatgcatgggtaaaagtagtagaagagaaggctttcagcccagaagtgatacccatgttttcagcattatcagaaggagccaccccacaagatttaaacaccatgctaaacacagtggggggacatcaagcagccatgcaaatgttaaaagagaccatcaatgaggaagctgcaggcaaagagaagagtggtgcagagagaaaaaagagcagtgggaataggagctttgttccttgggttcttgggagcagcaggaagcactatgggcgcagcgtcaatgacgctgacggtacaggccagacaattattgtctggtatagtgcagcagcagaacaatttgctgagggctattgaggcgcaacagcatctgttgcaactcacagtctggggcatcaagcagctccaggcaagaatcctggctgtggaaagatacctaaaggatcaacagctcctggggatttggggttgctctggaaaactcatttgcaccactgctgtgccttggatctacaaatggcagtattcatccacaattttaaaagaaaaggggggattggggggtacagtgcaggggaaagaatagtagacataatagcaacagacatacaaactaaagaattacaaaaacaaattacaaaaattcaaaattttcgggtttattacagggacagcagagatccagtttggggatcaattgcatgaagaatctgcttagggttaggcgttttgcgctgcttcgcgaggatctgcgatcgctccggtgcccgtcagtgggcagagcgcacatcgcccacagtccccgagaagttggggggaggggtcggcaattgaaccggtgcctagagaaggtggcgcggggtaaactgggaaagtgatgtcgtgtactggctccgcctttttcccgagggtgggggagaaccgtatataagtgcagtagtcgccgtgaacgttctttttcgcaacgggtttgccgccagaacacagctgaagcttcgaggggctcgcatctctccttcacgcgcccgccgccctacctgaggccgccatccacgccggttgagtcgcgttctgccgcctcccgcctgtggtgcctcctgaactgcgtccgccgtctaggtaagtttaaagctcaggtcgagaccgggcctttgtccggcgctcccttggagcctacctagactcagccggctctccacgctttgcctgaccctgcttgctcaactctacgtctttgtttcgttttctgttctgcgccgttacagatccaagctgtgaccggcgcctacggctagc

SEQ ID NO: 97 - DNA, 801 bp, synthetic construct
  source 1..801: mol_type = other DNA
gaattcgccaccatgctgctgctggtgacaagcctgctgctgtgcgagctgccccaccccgcctttctgctgatcccccagagcgtgaaagagtccgagggcgacctggtcacaccagccggcaacctgaccctgacctgtaccgccagcggcagcgacatcaacgactaccccatctcttgggtccgccaggctcctggcaagggactggaatggatcggcttcatcaacagcggcggcagcacttggtacgccagctgggtcaaaggccggttcaccatcagccggaccagcaccaccgtggacctgaagatgacaagcctgaccaccgacgacaccgccacctacttttgcgccagaggctacagcacctactacggcgacttcaacatctggggccctggcaccctggtcacaatctctagcggcggaggcggcagcggaggtggaggaagtggcggcggaggatccgagctggtcatgacccagacccccagcagcacatctggcgccgtgggcggcaccgtgaccatcaattgccaggccagccagagcatcgacagcaacctggcctggttccagcagaagcccggccagccccccaccctgctgatctacagagcctccaacctggccagcggcgtgccaagcagattcagcggcagcagatctggcaccgagtacaccctgaccatctccggcgtgcagagagaggacgccgctacctattactgcctgggcggcgtgggcaacgtgtcctacagaaccagcttcggcggaggtactgaggtggtcgtcaaa

SEQ ID NO: 98 - protein, 241 aa, synthetic construct
QSVKESEGDLVTPAGNLTLTCTASGSDINDYPISWVRQAPGKGLEWIGFINSGGSTWYASWVKGRFTISRTSTTVDLKMTSLTTDDTATYFCARGYSTYYGDFNIWGPGTLVTISSGGGGSGGGGSGGGGSELVMTQTPSSTSGAVGGTVTINCQASQSIDSNLAWFQQKPGQPPTLLIYRASNLASGVPSRFSGSRSGTEYTLTISGVQREDAATYYCLGGVGNVSYRTSFGGGTEVVVK

SEQ ID NO: 99 - DNA, 26 bp, synthetic construct
  source 1..26: mol_type = other DNA
taggaccgccctgccccccttgccct

SEQ ID NO: 100 - DNA, 330 bp, synthetic construct; identical to SEQ ID NO: 77
  source 1..330: mol_type = other DNA

SEQ ID NO: 101 - protein, 25 aa, synthetic construct
LEGGGEGRGSLLTCGDVEENPGPRM

SEQ ID NO: 102 - protein, 356 aa, synthetic construct
LLLVTSLLLCELPHPAFLLIPRKVCNGIGIGEFKDSLSINATNIKHFKNCTSISGDLHILPVAFRGDSFTHTPPLDPQELDILKTVKEITGFLLIQAWPENRTDLHAFENLEIIRGRTKQHGQFSLAVVSLNITSLGLRSLKEISDGDVIISGNKNLCYANTINWKKLFGTSGQKTKIISNRGENSCKATGQVCHALCSPEGCWGPEPRDCVSCRNVSRGRECVDKCNLLEGEPREFVENSECIQCHPECLPQAMNITCTGRGPDNCIQCAHYIDGPHCVKTCPAGVMGENNTLVWKYADAGHVCHLCHPNCTYGCTGPGLEGCPTNGPKIPSIATGMVGALLLLLVVALGIGLFM

SEQ ID NO: 103 - DNA, 321 bp, synthetic construct; identical to SEQ ID NO: 78
  source 1..321: mol_type = other DNA

SEQ ID NO: 104 - DNA, 66 bp, synthetic construct
  source 1..66: mol_type = other DNA
atgcttctcctggtgacaagccttctgctctgtgagttaccacacccagcattcctcctgatccca

SEQ ID NO: 105 - DNA, 735 bp, synthetic construct
  source 1..735: mol_type = other DNA
gatatccagatgacccagtccccgagctccctgtccgcctctgtgggcgatagggtcaccatcacctgccgtgccagtcaggatgtgaatactgctgtagcctggtatcaacagaaaccaggaaaagctccgaaactactgatttactcggcatccttcctctactctggagtcccttctcgcttctctggttccagatctgggacggatttcactctgaccatcagcagtctgcagccggaagacttcgcaacttattactgtcagcaacattatactactcctcccacgttcggacagggtaccaaggtggagatcaaaggcagtactagcggcggtggctccgggggcggatccggtgggggcggcagcagcgaggttcagctggtggagtctggcggtggcctggtgcagccagggggctcactccgtttgtcctgtgcagcttctggcttcaacattaaagacacctatatacactgggtgcgtcaggccccgggtaagggcctggaatgggttgcaaggatttatcctacgaatggttatactagatatgccgatagcgtcaagggccgtttcactataagcgcagacacatccaaaaacacagcctacctgcagatgaacagcctgcgtgctgaggacactgccgtctattattgttctagatggggaggggacggcttctatgctatggactactggggtcaaggaaccctggtcaccgtctcgagt

SEQ ID NO: 106 - DNA, 36 bp, synthetic construct
  source 1..36: mol_type = other DNA
gagagcaagtacggaccgccctgccccccttgccct

SEQ ID NO: 107 - DNA, 84 bp, synthetic construct; identical to SEQ ID NO: 5
  source 1..84: mol_type = other DNA

SEQ ID NO: 108 - DNA, 126 bp, synthetic construct; identical to SEQ ID NO: 6
  source 1..126: mol_type = other DNA

SEQ ID NO: 109 - DNA, 1074 bp, synthetic construct; identical to SEQ ID NO: 9
  source 1..1074: mol_type = other DNA

SEQ ID NO: 110 - DNA, 48 bp, synthetic construct
  source 1..48: mol_type = other DNA
atgcttctcctggtgacaagccttctgctctgtgagttaccacaccca

SEQ ID NO: 111 - DNA, 753 bp, synthetic construct
  source 1..753: mol_type = other DNA
gcattcctcctgatcccagatatccagatgacccagtccccgagctccctgtccgcctctgtgggcgatagggtcaccatcacctgccgtgccagtcaggatgtgaatactgctgtagcctggtatcaacagaaaccaggaaaagctccgaaactactgatttactcggcatccttcctctactctggagtcccttctcgcttctctggttccagatctgggacggatttcactctgaccatcagcagtctgcagccggaagacttcgcaacttattactgtcagcaacattatactactcctcccacgttcggacagggtaccaaggtggagatcaaaggcagtactagcggcggtggctccgggggcggatccggtgggggcggcagcagcgaggttcagctggtggagtctggcggtggcctggtgcagccagggggctcactccgtttgtcctgtgcagcttctggcttcaacattaaagacacctatatacactgggtgcgtcaggccccgggtaagggcctggaatgggttgcaaggatttatcctacgaatggttatactagatatgccgatagcgtcaagggccgtttcactataagcgcagacacatccaaaaacacagcctacctgcagatgaacagcctgcgtgctgaggacactgccgtctattattgttctagatggggaggggacggcttctatgctatggactactggggtcaaggaaccctggtcaccgtctcgagt

SEQ ID NO: 112 - DNA, 357 bp, synthetic construct
  source 1..357: mol_type = other DNA
gagagcaagtacggaccgccctgccccccttgccctggccagcctagagaaccccaggtgtacaccctgcctcccagccaggaagagatgaccaagaaccaggtgtccctgacctgcctggtcaaaggcttctaccccagcgatatcgccgtggaatgggagagcaacggccagcccgagaacaactacaagaccaccccccctgtgctggacagcgacggcagcttcttcctgtactcccggctgaccgtggacaagagccggtggcaggaaggcaacgtcttcagctgcagcgtgatgcacgaggccctgcacaaccactacacccagaagtccctgagcctgagcctgggcaag

SEQ ID NO: 113 - DNA, 687 bp, synthetic construct
  source 1..687: mol_type = other DNA
gagagcaagtacggaccgccctgccccccttgccctgcccccgagttcctgggcggacccagcgtgttcctgttcccccccaagcccaaggacaccctgatgatcagccggacccccgaggtgacctgcgtggtggtggacgtgagccaggaagatcccgaggtccagttcaattggtacgtggacggcgtggaagtgcacaacgccaagaccaagcccagagaggaacagttcaacagcacctaccgggtggtgtctgtgctgaccgtgctgcaccaggactggctgaacggcaaagaatacaagtgcaaggtgtccaacaagggcctgcccagcagcatcgaaaagaccatcagcaaggccaagggccagcctcgcgagccccaggtgtacaccctgcctccctcccaggaagagatgaccaagaaccaggtgtccctgacctgcctggtgaagggcttctaccccagcgacatcgccgtggagtgggagagcaacggccagcctgagaacaactacaagaccacccctcccgtgctggacagcgacggcagcttcttcctgtacagccggctgaccgtggacaagagccggtggcaggaaggcaacgtctttagctgcagcgtgatgcacgaggccctgcacaaccactacacccagaagagcctgagcctgtccctgggcaag

SEQ ID NO: 114 - DNA, 84 bp, synthetic construct
  source 1..84: mol_type = other DNA
atgttctgggtgctggtggtggtgggcggggtgctggcctgctacagcctgctggtgacagtggccttcatcatcttttgggtg